European Patent Application EP 4 755 903 A1, published June 10, 2026. Title: Genetic Constructs for the improved Expression of Mureidomycin A. Applicant: Eberhard Karls Universität Tübingen. Application EP. The sequence listing filed with the application follows.

SEQUENCE LISTING (3 sequences)

SEQ ID NO: 1 - DNA, 42055 bp, synthetic construct
  misc_feature 1..42055: note = Cosmid containing gDNA of Streptomyces coeruleorubidus AB1183F-64
  source 1..42055: mol_type = other DNA
gaattcgcggccgcaattaaccctcactaaaggatctctgttcgaggctgccgttcgtggcccaggtggtcttcgccgtgcagcggtccttcaggtcggtcctcaggcgcatcgtgaccgtgccgttggtgtcgttgtccggggtgttgctcatgtcgacggtcaccgaacgcagtgcgcccatcgtgtcgttggcctcgtcgagcaggtccgccggggacttctccgtgccgccgccacctgccccgcacccggtgagcacggctgtcgtgagcagacacgccagcgctgccgtcatgggtgtcgtccgcatcgaggccccccgcccgtttccccatcgagggcctcgtcccacggaatcggaacaaggccctgaactgcgacgacagtctaccgaagggccggacgacgaaagccggtaccgatctaggcctggggagcgccgttctccacatactcgtacaggaatgagtcatagaactccgcatccggagacggcacgatctcgaccagattccagtgggcccgcatctccgcggctgaggctgccaccggggtcttctcgagatcgctcccctgcccatccggctgacccctgccggtaaagcagagcaccacgttgcgtggatgccgtcggacagagtcctcgattctttccagaacagccagggacacgtccaccgaaaagggctcgtagaaatagaagagccccgcatcgtccggaatgtcgaattttgtggcatcagcatgcaccacttcaatacggtcgcagccgtcgcgggctaccgaagccttctccacgttactccgggcaatgtcacagagagcttccgatgcctccacgccgacgatccggcgaaagggaagctcagccgccagcaacaggactcgacccttaccgcaaccgacgtcgacaaacgtcacttcctcatgcctgacgtcgcatttgccgagcgcactgcgcacggtacggaccggcgtcggcgagtacctggcgtttcgccctacccacagctgatccgcgtcaggaagatcccacagttcgacagattccgtggtgtcaacgtcgagaaccgagtcaaacggcgtttcctgttcgattcgaccgagccgctcatcaaattgctgtcggtactccatggcacgcaacagccttgcccgagcatcattgtccgacatcccgtcaccctttctcgatcagaaaaaatgcctggtttcgaaggccggccgcgccttcaaagaagtcgtcattgcggccgacactcgacgtcggcagatcgcttttgcctggcttccgtcgccttactgatgccgacgccttgcattccggggatccgtcgacctgcagttcgaagttcctattctctagaaagtataggaacttcgaagcagctccagcctacaaaaccttgcgaacccccggccttcggctgcgaaatgattctgcggcgtgctggttgagctcctatttccgaacaatagattagcgatcggcgcaccgaactgtactgacacccgtcaggtgcatcggcctcttgtatttcgaagaaccatcggcatttgcggttcagctcgcctcgcgtaccacgtccgccacgatcgccactgcggcggagacgtccgccgagctgagaccgcgatgtgtgacggccctgatgcggccgtggccgaattcgcccatcaccagcccgcgctgctcgactgcgcgcaggaagcggtcgtcgtccagcccgttggccgtgacccggaacaggacgatgttcgtggtgaccgagctcgggtcgacgtcgatcccgtccacctccgccaggcccgccgccagttgtgccgcgcgctgatggtcctcggcgagccggtcgatcatggaggtcagcgcgaccagccccgccgctgcgaatacaccggcctgccgcatgccgccaccgagcatcttgcggatacgccgggccttctcgatgaagtcggcctcaccggccaggatcgaaccgatgggtgccgacaggcccttggacagacagaactggatcgagtcggcgtgggcggcgatctgctccgctgccacgcccgtcgccacggcggcgttgaagatcctggcgccgtccatgtgcaccgggatgccgtgcccggtggcgaagcgcttgagctcagccagatacgcctgactcagcacccggccccccatccggttgtgggtgttctccacacagatgagccccggcagggcgaactgagggtcgtccgggtcgggcggaaaggccgcggccaggtcatccagcgcgagagtgccgtcaggccgggtgggtatcggctcgtagacgatgccgccgcacacgctcgccccgccggcttcgtacaggtagatgtcgctctcgttgccgacgagcaccttcccgccccgcggcacgtgcaccaggagagcagcgaggttcgccatcgttccactgggcatcagacacgcggcaggcttgccgacgctcttcgcggcgagctcctccagccggttggccgtcggatcctcgccgtacacgtcgtccccgagcactgcctgggtcatcgccgacaccatctgctcggtcggcagcgtgaaggtgtcgcttctcatttcgatcaggtcagccatgtcagcccgtccctcgctcagtcgttcgccaaccggacagtgatggagtccagcgccgaatcgagcgactggtcgagctgcgagaccgagtcgcccgaggcgatgatgtaaccgatccggtcgtaggcgtcggtggccggacgtaccgggtcgcccggcctacgcgcgatctggacttcggcgacaccggccgactgccgggccgactcgacgccgtccaggctcgccagccgtccttccgcggagctcgtgatgaaggcgactccggtcggggtcagcgctccccgcggtagttcgacggccatcccggccgccgcgcgcagctgctgggtcagcaggtcgggcccgccggccagcctgatcagctcgggaatcatgccgcccgcgagccgggcgttgatctcgatgatcgtcggccccgccgcggtcaggcgcagttcggtgtggcaggcgccgtgacgcagcccgatcgcctggatcgccgcccgtaccacctgctcgatctcgcgggactcagcctcgtccagtgaggccgggaaggcgtgccgcagctcgacgaacgagggagggggcgacaccgacttccgggtgatgcccaccaggtggagtgccgcgtcgacgaagatcgtctccacgctgaactccggtccctggacgagttcctcgaccagcacctccggcgggacggcctgctcacgcacgttgtgcgtgatcgcgagcagcttcgcggcgtgctcctgggcctgctcgacggaggtgcacagcaaaactcccgtcgacgccgagtccgaggccggcttgaccacgcacggcaggcccgtggccgcgaccgccccgggcacctcggccacccgcgtcacgggcatcgagaccggctggggcagtcccgcgtcggccagcagccggcgggttgccgacttgcggcggcacgcgcccactgccgcgggcggattgccgggcagaccgagcgatgcggccagcgaagcggcggcctccaggtagaactcgctggtggtcgtgatgccggccacctcgtcgggggcgaagtgggctcgcagggcggccgccagcgtgtccgcgctgttggtgtcgcagcggatgatctcgcagtcggcttcgccgatgccggggtaccggctgggccgactggtcagcagcacaggtgccaggccgaggtccctggcgcgcgcgagggcgagcattccggtgcccgtggtgttcgactcgacgaacaccaggcgcttgcgcggcgtggacggcacctcggcccgcgcccagctgctgacctcggtgccgtaactcacctccaacggctcggtccggagggggagttcggcgaggccggcctgctgccagtagccgtcgtcgtagatcgagtccacgtatcggtcgccccggtccgggaagatgccgacgacgcgcgtgccgggtgcgacggtggcggccaggtgcttcagcacctggtagaccgatcccgaggagttcccggcgaagatgccttcgtcgcgagcgagatcacgggtcgcgacgaaggcctcccggtcgttcagccagtggatctcgtcgatgtgggcgtagtccaggttgcccgggatcaggctgttgccgatgccgctctgcttgcgtcccggctggtccggctggccgaagaggacactgccgacggcgtcgacgccgatcacccgcagcggaccgtcgtgccccgccgccttcagcgcccggcgcagggcacgggcggtgccgcacagcgatccgccgctgccgaccgcgccgacgagcacgtcgatcctgcccagatccgccaccagttccccggccagtgcggcgtaggcgagcgggttctgcgggttggagtactgccgcggccagaacgcccccgggtactccgctcgcagggcggccaaccgctccagccgggcactctgccagccgttcgaggtcatcccctcgaccacatgcaccgagcagccgagtgccttcagcttcgcgagcgtgatcgcgtcgatgcgggggtccgtcacgatgtgcaccggatgaccgagcgcgtggcccgccagggcgagccccagcgccatcgtgcccgaggagctctcgatgatcggcgcgccgggggccagcaccccgttctcgcgagcctcgcgaatgacctggcgggcgacccggtccttcatggcgaacagattctgcagctcgagcttggccaccaccgtcacatccgtgggcgccgcccgcagccgcacggcgggcgtgtgcccgatggcgtcgacaaggtcattgaagatcattacttggtccgcttcctgtccgctcgaaacccaaggtctggtagcagaggacccgttcgcggtgcacgagctgaccgcagcggttgatggcctcggccagtcggctccgaaaccccggtacgtcatgcgggagcatcagcccgatcgtcgacccgctgtgcgcggtgaccacaccgaccccgccgatctcggcgctgagggcggtcatcgcgttcagcgtccgcttgcggcacaggcgctggttgaggtgggcgctgcgggtcgccacccggccgatcgcggccgcgtcaccggcccgcaccgccgtctggacctcgtccagcagccgggcgtactcctcccgctccgctgccgtgaagttcttgggaatcctgttgaacgcgacggtgtccacggtgccgccctcgtcgatgcccacgatggtcatcggcggcaggacgccgcatcgggccagcagcgcgacattgcggtgctcgaacgccacgactcccggatacatgacgccgtccgtcggctcgatccgacgcagcaggttctcgatgccctgcggcggcagatcgacgccgaccgcactggccaccgcccgcgccgtcgccacgagatcggccgaggaactcgccaggcccttcccctccgggagcgagccgctcagcctcagcgatccgccgccgccggagtgccgggcgagcacggcctcggcaaccctgcgggccttcgtcttcgtggccgggaacacctcgacgcggtcgtgtgcgctctcgtactcgaacgtcgcggtggcccacctggcgatgggcagggtgaccaggaagtcgggcccgtcgtcgggcagcgcgccctgcaacaactccccgaaggtgccgaaggccgagctgacggcgacggcccgagcgggagacccgtggtccctggccggctgctggacgagctgccggctcgtcatacgactcccccggccgtgggccgcacggcggcgtcggtggccgcgatcgcgtcccgcaccgttgccgtgcgtgcgttccactccgccgtcagcgcgtcgagccgctgccgctgctcggccagcagcgccaccacggagtcggggctggccgagcccgcggacaccttcgcgcgcagctgcgcgtccacgtccacggagttcgtcaggtaggaggcggggtcgtccagcggatagcccgcctcccgggctgccgagtcgagtgccgccgggttgctgtgcccggcgcggccgtcgccttcggccagcacggcggtgacgtacctgccggcgatgacctgagcggtccgccacggtacgccggcccgcagggtcagttcgttggccaggctgaagccgccgaagtgatcctcttcgcagaccgcgcgcatccggtcggtgcgccactgaagcttgtcgacgaccagggtgaatccggtcagcaccgcgcggatcgcaccgaacatcgtgctcgcgtgcaggcccgcctccttggagacctccaccatgttgctgtacggcgtgttccgctggccggtggcgaagtcgacgtagaaggcagtcaggtggccggtgcgtccgcgcaggcgttccagcagcgggtagttcttcttctggggcatggccgcggagatgccggccagctcgtccggcagctcgaccaacccgtaggcgctcgacgaccacgccatgaggtcggtcaggaagcggctgaatcccacgcccgcggaggcgatgtcggcggcgacatcgagcagccactcccgcgaggcgaccgcggccagtgcgtgcgggaccgggccggcgcagccgatcgcctgcgccaaccagtcccggtcccatgccagttcctggccggccatgggcccggcaccgagctgcgagaagttgatccggtcgtaggtgccgagcagccgggacgaggcgcgcagcgcgtgttccaccacggcgctgaggtagaagcccggagtgatgatctgcgccgactggaggtgcgtgtacccgggcatcggcgaggtgacgtcgtgggccgcccgctcgtgcgcgacctcggccagctccccgagcatggccgcgatctcgctcacctgctcacggccgtacagcagttgggcgcaggcctggaggtcgttgcggctccggtcgacgtgccaggccggcacgggctccgggagtgccttggcgacccgggtctccatcgccagcgcgatgtcggagagagcggcgccggcaccggcggtgagctcctccggggtcagcccgtcgagcgctcccgcgagctgttccacctgacgggccgacaggacaccgagacggtggtactcgcgcaggagcgccttctcgatcagcacataccagcgcagcaggtgggcgacttcgtgccggaactgcggctcgaggaactcctgcctgatgaagtcgtcgggcgctgccgcaagtcgaccggtcagtctcaccgggtgccgccttcctgggtggccgcgatggccgttgtgacgagatccgccgccgcagcggggtggctgcggacgagatagcgacccgcgtcctcgaaccgggtgatccgggccgcgggaagcactgccgcgcagcgtgccgcgacatcgctctcgcccggtgctcgcgggatcgtgatgatggtcgcgggcaggtcgagggttccggcgaaggcgccgagatagcgttccgcctcgccgagatcatgcaggtaggcgcgctcgatcagctcgccgcgggtcgacctccactggtcgacgtcggtgagcgcgccggcatcgcgcagccaggcgccgacgtcggccgagccggcggcggccggttcgcggtcggtggcctcccgctgttcggccgcggccaggaacaggtgccggggaggcactccggcggcttgcagcgatcggccggtctccagggcgagcgccacgccggcgccatgtccccacaacgccacggggatctcgatccggtcgcggatctcctgactcaaccggccggcgatccggtcgaggccgaccagctcgtcgtccggccgggcgacgtcatggccgggcaactccaccgcgtacaccgccacgtccgacgcggacagcgcccgtgccatggcctcgaagttgagcgcgttgcccgcctcgtacggcacgcacaccagagccacggtcgcggtctccggcaccgagagtgcctgcagcagcggggaatcacccgagtcggctccgtcggccgcggcggccaggtcggccagcaccgggtgcgccatgagatccacgagcgagatgagtccgccgagctgcacgacgagccggactcccgccagcgagccgccgccttgtgcgaagaagtcgtcgttgcggccgacctcgtcgagcggcaggcccagcacctccgcccacgcggtggcgatccgccgttcggtggcggtctgcgggggcgtcaggctgttgccgctcgcactgttggtctcgagatctgccagtccccgcttgtcgaccttggcgttgtcggtgagcgggagctcgggcagccagcgcagcgtacgcgggaccaactggagtggcagcagctcggccagcaggtcacggacggccgggatcggcgccgcggcggtgtagaagcccgccaggcgcttgctcgcgccgtccggcatcacgatcacacacgccgatcggacccccggcacccgcaggagctgggcctcgacttcgccgacctcgacccggaccccgctgatcttcacctgctcgtcccgccggccgacgaaccggagccgtccgtcgggcagccagtgcccgtagtcgccagtgcggtagcgacgcaggccggggcggaccggatcctcgccgaacgcctccgccgtgcgctccggatcgttgatgtagccccggccgacacagacacccgagaacgtgatctccccgatcgtgtcgtcctgcaccggcagtccgtccgcgccgatgacgtcgacgaggacgttggcgatcgggacacccacggtgacctggtcgtcgtccgccatggtgcggatgacctcgtgcgtggtgtcgtccgacgcctcggtggcgccgtaggcgttgaccacgggcacgccggggcactgcttgaaccaacgggtgagcacctgctggctcactgcctcgccggtgacaccgagcatccgcagtgagccgggcgcccggtccccccgctccaacctggtgacgatcacatccaggtaactcgggacgagttgcaggacgccgacgttctccgcggccagcagccgaaggagcgcggggacgtcgagcatcagttccggatcgatgatcacggtgctgccaccgacgatgagcggcgcgatcgcctgccatagcgagatgtcgaagcactgggacgcggtctgagcgacgaccgtgcccgggtcgagctcgaaggtgtccacctttgccagcaagtggttgagcatgccggcgtgttcgcaggcggctcccttcggcgcgcccgtggagccggaggtgaagtagatgtaggcgagcgcctggtccgggacacggctcggccgtgcttcgacggccgccaccggcaccaaggggagcgcgtgaacggccgcggcctcgatggggcgcgccgatacctcgtcctcgaccagcgccagttggctcccgctgcggcgcagcaggtcggcgatgcgctcgtcggggtacgccgggtcgatgggcaggtagaccccgcccgccttgaagatgccgagaatcgcggccagccagtcgagcgagcgctggctgatgaccgccacgacgccctcgggccgcagtccggccgccaggagtgccccggccacccggtccgcggcggcgtcgagctccgcgtaggtccagcgagtgccgcggtgcacggcggcggtggccgacggcgcgttgcgtgcgcactcctcgaagagctcgtgagcacggcggtcagggagtggccgtaccggcccgactccgcgtgactgctgaccgcggactgcctcgacctgctccgtcacagtgccagcctttccggccgaacgtagtggcggcctggattccagaacgtaactgactcgaataatgcaacgtgctgtggagcgttatggaagaccggtgcgacgagccgccggacttcgcaggtgcccgctatcggagcgaccctttcatgagcctcgtggtcgatcggaatcgatgcgcctgcgcggcgggcaccgtgccgctcggatcagttcggcgggacgtgcgatggtcgtcggctgtgtagcgatacgcggccccgcggcaattggcctctcatgaggaacaggctagtgacctgcggggttcacccgtactgacatcggtcagggctcgggcggctcggccgccaacggtgcggccggcgcccggatcgagacctacgcagccgcccggagacaccgtcacaccggagctccagcggtcgaccgccggtgccgccggtcgccgcgttccggccgaagtgctggcaggcatcggtacggtggcaccgtcgacgtacctgtatacgcgccatcctgaacgacagatgaatcaggggcggggagctcgacgcggagttgccatgtcgtgcacagcgcggcggtccagcttgcctgagtccgtcgacggcagctcagggacgaactgatagcgatccggcgccatgaagggcggaagggaagcgagcatgtgctgccgcagcaacgcctcgggcttttccggtgcttggtcggcgagcaccacacacgcggtcaggaactgggcgccggcctgggtgtcgaccaccgtggcggcggcttccctgaccatcgggtgggcacgcagatacgtctccacctcgccgagttccacacggatgccacgcaccttgacctgctggtcgttgcggcccaggtacgcgaaggcgccgtccggcagccgtctggccaggtccccggtccggtagtagcgcaccggcccctgcggagtgtcgaggacgacgaagcgttcggctgtcagttcggggcgccccaggtagcccacggccacgcccgagccggctatcaccagttcgccgacctctccgtccgggaccggctccatggcctcgccgcgtacctcgacgagcaggtgcggcagcgccgtaccgatcggtgagggcacggggccgtcgaagtcttcctgggtcagcacgcgacaggtggcgacgcaggccgcctcggtcggtccgtagatgttgacgacctcgggcggcgtgcccgggcagcgcgcgaggaaggcggagacgacatcaagctccacgctctcgccgcccaccaggacgtaccggagggcgaggggaggccggcccgccgcctcgtgggcgtgggcgagcgcccgcagcgtcgtggggacctgtatgacgagggtcacggcctcgcgtcgaagcaggtcgaggaagtcgggcatcgactgcgccacccgggccgggacgacgacggccgtcgcgccggccgccagggagagccagaactggaggacggacccgtcgaagatgaacgggaggaagagcccgacgcggtcctccgtgtccaggtcgaccaccgacatcacgccgcggaccaggtcgaggacgctggtgtgctggaccatgcaccccttgggcgtgccggtcgagccggaggtgtagatcacgtacgccaattcgctgccgtcgagggggacgggcggcgccggcgggatcgtctcctcggcctcgggggcgaggacacggacatccttgagcccgccggcagcgcagtgcccggcgtcgccgacgaccaccccgatgtcagcgtcgcgtaccaggaagcgcaaccgctccgccggataggaggggtcgagcgggacataggcggctccggccttgaggacggccaggatggagatctgcgtctcggccgagcgtgggaggaggatccccacccggtcgcccggtcggaccccttccgccgccaggcgtgcggcgatccggtccgtcaggtcgtcgagctcgcggtagctgagggtccgctcgccgtctcggagggccggggcggcaccacgggccgcagcaacagcgcggaagagatcgggcagggaaacggccgtgtcgagcagagaccgctgctctgcggcggtcataggtttgcctctcagagtttcaggatggctcgacgcttccggcgccgcttgcaggccgccattgcacaggcggaaggatccaccctctccgccctgtccgcccgtcagcgaggcggcgtccgcgacgacctgcgggtggtgtcgctgcccccgtagtggcagcaacctcctcggctgtcgtgcaaccttcggcgcgatgactaccgccttttatggagcgtcagattacgtatcgcgaggcggtgcttgtactgacagcggttaggagaccatggccctgcgttggtgttagatcgggtagcactgcccctgacctgtgtgaggcatgcgcggtcggccggcgggccgacgaccacgctggtgcaggcgtgcgtggcgttggcctcgacgcggtgggagtttgcagcgccggtcaccctcgcgggcgacgatcgaggctcccgcgcccatgtgccccgtcatcccaggtcatcaggtcatgcggtggatccaggctgacgtactgacaggtatcagtaccggaataccacctatgcgcctgcatactcgacgctagtcgtatcaaaaaggagacccggtgtgtttccgctcagcgccgcacagcaaatcgtctggctccagcagcaggtgcttccggagagccgcgcctatcacgccaccgcggtggtcgaatttcatggtgaattcgatccggtggtgatccgccgatgtatcgccgacgcggtcggccgccacgacgccttccggatccggatgtgtgacaccgattccgggatccccgcgcaggaggtcgtcgcggatatctccgtggaggtctcccagtacgacctgcgcgacgccgacgaccccgcggtacggcggggggaactgctccgcgggcaggtcagcaccgccttcgacctacggaccgcgccgctcgtccgctggatgctgctgcacctggccgacggtcactggcaactcgccatgaccgaacaccacctggtccacgacggccggtccaccgtgatcttcctcggcgacgtgctcgaccagtacgcggccgagatgtccggcggagaccacgtcccggaggctgccccctcgtacgaggagtacgtcgcccacacgggctcggacgagtaccgtgcgcgggtcgccgccgacgtcgcctggtgggcggagcggctcgacggtgcccggttcagcatcgacttccccaccctggggacccggcgctcggccctgttcgatcaccgcggcgggcagttccggcaggtgctctccgccccgctcatggaccgggtgcgggatgtcgcccaggagagtggtcacacggtcttcgccacgctgcttgccgtctactccgaactgtgccgccgccactccgggcaggacgaactggtcatcggcatgccgctggccaaccgcccggtggagttcgagcacacggtggggatgatggtcggcgccgtaccgcttcggctggcgatcgaccccctggctccgggcagcgacctcgccgaggaggccatgacggcggtcttcgacgccatcgaccatgagtcggctccgatccaggacctggtgacggcgctcaagcgcagcagcaaagggctgggcaacccgcttttcaacatcatgttcgccatgcacgacgccccctgtccgcccgtgaagatccccggcctctcggtcaacatggagatcgccgtgagcgccggcagcaccaagttcgacctgagcgtcgtggtcatgccggacaaggtcctgcaggcggaccacggcgaccacggctacgaactggtctgggagtactccactcagatgttcgggcccgaggacgtggagacgctcgccaccggattcgagaccctgctccgcgcctacgtcgccaggccttccgcgccgatcggcaccttggcaccggccgtggccgcgcgtccggcacgcgacgcccgcgacaaggacgaggagttcggtgcggcggaggtggcgccgcgcgccggggacgctccggccaccgacgccggaacgccttccggctcgctgtggctgcaggcgttccggcacatcctggagcgcgacgacatcgacgaggacaccgacttcttccaggcgggcggctattcgctgctcgtgccgctgctggtggcgcactacgagacgctcgcgggccgacggactccgccgagtctggtcttcgagttctcgttgccgcgagaactggaggcggcgacggccgcgatggcggggcgctgacgacgagctgaaagaaaatgaccaagtacaaatacacagtcgaagaatcggaaagattcaacaagcatggcatcgacctgactgtttacggtcaggtcgatccgtcggcgacagtcgttcgtgtgagtgtcgagcgcgggcactttcaggaattcttcaatgtgaggagttcctatacctattacgtcgtcagcggccagggagtgttctatttgaatagcgaggcggtccccgccggcgccactgatttgatcacggtcccgccgaacacccgaatacactacttcgggtcgatggagatggtcctgaccgtggcgcctgcattcaatgaacaagatgaacggcatgtcaggttcatcagtgaaagcgagagcccttactaatgccggtaccgccgtggcggtgaccgagtacgtgatgcctctcggcctattcctcatgggagcgggcatcaccaccagctggatggaggatggcatggaggatggcaagtcgatgaccacggaccacgccgcactgcccacggggtgccacgcgcgcactccggctccgccgccggacgcagcgtccctgccggacgatccgcccctgccgcacgaactcgccctgccgacggaccggtcgcggccggcccaccccgcgccggccgtggagctgcaccggttcgacctgactcccgggatccaccgtgccctgctcgccaccgccggggccgcccgggcgtcgctgcctacggcgctccatgccgccgtggccgctctgctgacccggctgggggccggcgtcgacatcccgatcgcggcaccggcggactccccggcccggtacctcagcctgcggatcggaacagacggggacccgagccttcgtgagcttctcgtacgggctcgggaggcgggtcgcacggcccgcgcgaggcaggacgtcgccacgcgacgccggacggacgacgccgacccggtgcggcgcgtcggaagcggtccggcggcccaggtggccgtgctcgtcgtcgacgagcacggccccggctgcgacccgacgggcacgaccggcttcgacctcgccctcaccgcgacggagcgacggggggccgagggcgaaccggccggcatcgcctgcgcactcgcctacgactccgagctcttcgaccccgggacggccgctgcgctggcggcgcgtctggtcacgcttctcacggcattcgccgacgtcccggacaccgcgctgtcgcgcgtggagctgttctccgacgacgagcgccgggcctggctggcgatgtccagtggaaccgagcatgcgatcggtgagtgcaccctggtcgagctgttcgagacacgggtccgggcgacgccggacgccgtggcgctggtgtgcggcgaccgttcgctgacgttcgccgaactgaacgggcgggccaacgccctggcccggcggctgatcggggcaggtgtccgctccgaggagccggtggccctcctgatggaccggtcggcggagcagatcgtctcgatcctggcgatcctcaaggcgggcggttgctacctcccgctgcacctggcgcatccggcgcgacgcatgaccggcgcccttgaggctgctgaggtcaggatcctgctgaccgatggttcgcacgccggccacgaggtcgcgagggccgccgggacgacactcctcgtgacggcggacggtccggccgcggcggacggcggtgacctcgaccgcaagccgctgcccgagcaggccgcgtacatcatgttcacctccggctcgaccggcacccccaagggcatcctggtgccccaccggagcgtggtgcacctggccctcgacagatgctggggcgaaggcgtgctggagcggatgctggtgcacttctccgccgcggtcgatccgtcgacgggcgagatctgggccccgctgctcaggaacggcagtctggtgatcgcaccgcccggcgatatcgacgcgcaggagctgcgggagctcgtctcccgctacggcgtcaccggcgccatcttccccggcgggctcttccggatgcttgccgacgacgacccggccgcgttcgcggggttgaccggcgtctacacgggcggcgaggtcatttcgccggtcgcggtgcgcaaggtgctcgacgcggctcccggtctcctcgtgcaccccctgtacggaccgaccgaggcgaccctggccgttacctaccacacgattcggcaggcaggggagctggcgggagatgtccccctcggccggccgatggacaaccggcacgtctatgtcctggacgagcatctcaacccggtgccgcccggcaccgtcggcgagctgtacctcggcggtgcgggcctggcccgcagctacgtcggcagcccggttctgacggccgaacggttcgtcccggatcccttccaaggggtgggtgcccggatgtaccggtcgggggatctggcccgctggacgcgtgacggcgtcctcatgttcgtgggccgcaccgacgagcaggtcaaggtacgcggctaccgcatcgagctcggggagatcgagaccgccctggcccggcaggaaggcgtccggagggtcgccgtcgtcgtccgggaggaccagcccggcgacgaacgactggtggcgtacctggtgccgggcgcgggagcggcaccggacccggaggcgctggccgaggagctgcgcgccactctgccggcgtacatggtgccctccgccttcgtcgccctgccggagctaccgctgacgccgaacgggaagacggaccgtacggccctgccggcgccggactacggcggcggcgcgggccaaggcccccgcacggccgacgaggagcgtctgtgcgctctgttcgccgaggtcctgggggtggaacgggtcggcgtggacgagggattcttcgccctgggcggggactcgctgttggcgacccggctgaggaccaggattcggagcgcgctcggtgtcgacctcagggcgcgagtgctgttccggcacccgaccgtcgccgagctcgcgcggctgctctgacctcgtgccacgcgtttgcgatggaaaaggcgccgccccggtcggggtggcgcctttggcaggtgcggtccgcgtgggaccgcacctgaagcggtagtaactggagctacgggaacacgggttactgcacgggggtgccgaggtagccggggaagcggccttcggggtcacggacggtgcggatctgctggaacttcgaccaggccgcgtcggacatgatccggtcggggcggacggtgaagtcgctgtcgcccaggtagcagccggccgagtacggtgccgcgcgctccatggtcccgtccagccaggagcggcaccgggcgtcctcttccggggtttcgccgatcacgtacgcggcgaagtacaggtcggtctgcaccgacagggccatgtccggcgggcggcgggacagcaggggggtgaagtcgcccaggaccgtgaacgtcttggacgtcggcagatcggtgaaggcgggcaccagcgccggcaccacctcggaggtggggccggagaggaaggcgttgtccgcgaaatagcggtggtagtcggggttggaccgcagttgatcggcctggaggtcggcgaactccaccggctgggcgaccttggtcaccagggccttgtcgacgactggacaggtgccgagcgcggccggcgaggccgggccgccgtcgaacgagaccgcgtcgatgatcagcaccggcgagtcggacccgggcggagtgcagccgacggcggcgagttcgacggacggcggcaggtcgtggcgcgccgcgtggtaccaggtcaggacctccgaggcgagctcggtgggatagacgtaggtggagcgggtcagctcccggaaccgggggcgggtacgcagccggaactcggtgaccacaccgaagaaccctggacccgacccgcgcgccgcccagaacaggtcggcgttctcggtctcggagcaccggaccagctcgccggcggcggtcaccacgtccatggactcgatggactccgcggcccagccccacccacggcagttccagccgatgccgccctgtagcaggaagccgcccatgcccacggtgggggcgtggcccacggcgaagaaccggccgtgcccggcgagatacgggtccaggtccaggccgccacgcaccgccggacccaccgccacggttgcgtcggcggggtcgtaggacatcccggtgaacagggccagatcgatgagcagggtgtcctcgcgcagcgaccaggcagcccaactgtgcccgccggagcggacggcgaccttccagccctctgccgccgcgagcttcactcctgccgccacatcagcggcgtgagcggcacgcagcaccgccgccggtcgccgcgacggccgccggtggttgaagacgcgcgaggtcgtggcttcggcgaacccggtgtcgccgctccgccagaaggccccggtgaaagcagtcatcagtacgcgatccccaagtcggtctgcacgccgtgcagatcagtaggcacacgtccgggctgctccagggccgcctggccgaacatgcgagtggatgtcggccaggtcgtggagttggcggcgagtcaggcgcgggatgccgccactgcgtgaccgatcggccgtcaggcggctgatccctcatcggcggacaggctctggcgcaggctcgcaggcctcatgtccgtccaggtacggtcgaggtaggcgaggcattcggccttcgggccccgcgtcccgacctcgacccagccggcgggcaactcccgcccggacggccagatcgagtactgctcctcgccgttccgcactacgcagaactcgcgcccctcgtcgtcgaacatgccactccttgagcgttccgtggccgacaccggcacggcgagcggttctcgcagcaccgtcggcagggtttcggggtttcggggtttcggggagcggttcgtcatcgcactgcctgcctgtgccgagacggcgaacacggcacctgattcatgcaccgggaccttcggatccgcgattcctctgggcgcttcgacggtctccctagctgccggcggacagtgcgaacctttcggccgcttcgaggaccttttccacggccgcgccggggaagtagctctcgttgtagtgcgcgacgagttccggccccgtctcgtacaggttccacgcgacgaccacggtctccacaaagcgcttcccgccggggaagtccagttcgacgtactccccctcggttccggtgaacgcccgcaggttgtatgtggacggcggttgttcgttgagactgacgtacagccccgcttgtttgtccgccaccatcagagtctcgttccagtaccttccggcgacgaggagcggaatgctgtactcgaagacgtcatgggttcgcaggaacacttcccggacggtttcgagcgggctcctggtctgccgtccgaggtgcagcgggacggtctggacaaacagcccggcggtctccgacgtgcccggcagcatgcgaccgtgttggttgacggagatccccgccagcggatcgccggtgacttcccgcatggcggcgagcacactggcggtgaccaccgcaaaaggggtcgcccgagcctgcagcgagaatttgtgtacctgcgacttcgcatccgccggaagttcacgggtgacacgcctgggttgatactcaccggtgtgctcggcgccgaccgaaaagggcggagggaacgtcccgaactccccgacgtaggagcgccagaacgctctgcgctcctccccccacgcgccggagaacaaacggcgctcctccgaggcgaaactctggtagctgcccacattcgtgacgtcgccggcatcgccgaccagagcacgattgtagaattcggtgaaatccgcccggatgcgggcccaggatgcctgatcgctgatgatgtgatccatcgcgatcccgaagagatgccttcgctcgccgcactgcacgatggcgatacgcgagaaccccgggccgtccaggctgaagggggtgccgatgaaccggcgcatcagctcgatcgcctctgcgtccgtttcggcggtgtggaattctacctcgctcagcgcgtcatcatacgtacatgcttcatccgccgaagcgtaggtccggcgcaggacgtcatgacgcaggcagacccgccaccacgcatcgcgaaccgcggcaatgttcagttccccggtaagccacatcgccatgtagtgcagattgtgccagtcggcgaactctccggtcagcctggccatttctgcgaacgaagtcggaccccgggatgtcttgacctgagacaatgtcatttcctggtgccgttcgcaccggtatccccctgccccagctcaccttccaggaaatcagaaaggcttcgcggtgaggtgtaggaaaacacgtgacgcagcttcacatcgacacccagagcatcatgaatcatgccggtgatctgcaggacgtgcaacgacgacccatcgttctcaaaaagatccgagttctcgtcgagatccggcttgccaagaaccttccgccagatctcggtcaggaccgcaacacgatccggcgccttctgatcctgtagattcatgtcgggagctcctcacgacttgctgcgcgattttctggtacgacaacttgcaggttgcggcggacccgtaaaaataccgatcggcaggatgcgcctgtactgacaccagtcaggatcatggcgacatcacctgcgcccgccgcgatcacgactgatgcgaaatctcatgtgctcgccgcacctgcgcactctcctgggcacccgtccttggacgcgaggccgcggccggggtcagtcgagccaggtcaggaagtgctccagctcctcccgcagttgagcgacggacggccgctgcacctcgatttcggtcttggtctgctcgccgacgggagacgtccggtagacattcgtgaaatcttccacggcaggcggctgcaggacgagcgacgccgcggccttgccggcagatcgggagatgcagtgcagcacctcgtgattgatgtggtacaccgttccggccggcaggagcgcctcgaacacgctggacaactgttccttgccctgtgcttccagggagaaggtcttcccctgcccgatcggcaggtacttgaagtggtagtactcggtgccggggccgatcttgaactcctgggcgaagtactcgccgaccacgagcgcggtcgtgaagtcccagcgatgcgagtggatgtcctccgtgatggtccccgaggcgttcggctgcggatgccacatgtggaggcgcagcctccaggggttcttgtcgccggccagcagcacgaccttcaggaagttgttcgcgtggtagtacgagcgggcggctatgtcggcgagggcagtgtcgtcagagatgatctgaccgatcagggaacgcagttccttcggctcggcaagatggcggaccaccgactccgagccctggaaagtcgtgccgcgcccgctgtccacgaccacttccaggtggtccttgatttcctgcagggtcgcttctgctagaacctgcgccatggcctgtatctccctttctggatgctggcgatccagcgacttgatgtttgtggaaaggcaagaccctgtgcaacggtcgccttctgctcttggggcctgcgaaccgatccggggtgctactccccgccgagggcgatcaggaattcaggggagccttcgaactgcgatcggccttgggccatgatgatgttgtcggtgatcagcaggtcgccgcgacgccacgggacaccgaccctcaccgagtcgtaggcgtgctgaatggcggtcaagtcctcgtcggacagcggcgatccgtcaccgaagaaggtgttcatcgggaggtatttcccgaaggcatcggtcatgatgtcgcgctcgaccggatccaggttgccggcgttgaggaaggagatctgattgaaccagcactcctccccggtcgtcggatgatcgatgaagccgggccggtggcgcaccgtgtacagcgtgccgttggggagccactcgggtttgattccggtggtctcgaaaagctcgtcgagtgctgcgcggtccgccacggagaacgcttcctgccacgtgatgccgaacccgtcgtggaaggacctggccatggtccagccacccgtgcggacacgatcggcgaggtgcgccggcagatgaccggctatccgacgggtgtcactgaggtgcgactgcccctcgccgtccggcggggtgatgcacgcggtgagcaccaccgaggggaacgtcctgctgaaggagctctcctggaacgggcaaatgacccggtcgttcggccagttgatcggtgagaatatgccgtttccgaagtcgctacggttgttgaacgcctcggtgggcgtgtggccggcgatgcccagggcatttcgcgccttggcaagactgtccggtccgtccatggggagtccgtggatgagaaccgctccccggagcagcatgtggtcacgaatggtcgccgccatgtcgtgcagccacgagaacggcgagtcgcccggggcatcgaaggaagaaacgagtacttcctgccgcatggggacggtctcgctcacttgatctcctcctacttgacttgacccgtccggaactcagtgagggtcatcgtcggtcgatgtctgaacgccggagaatcccgctcagaaccccggctccgccgaccccgccacccgccgcaccaagcgttcggttcagcgatgtgctgcggcggcgatgtcgacggcgccgctgatcttctggagcgcttccgccgtgtcgtcgtcggtgatcgtcagcgggggcgcgatgcggatcacaccgcgctcgtgacgtgtcatcactcccgcctgggccgcagccgccgcgatgtcggcagccgactccggactgtcggcctcgatggcgaccaccagtccgagtccgcggacatcggtgatcagcgggctcgactcgagcttccgcaggccctccaacagcgtggcgccctgggccgccgagttctcgacgagcttctcgtcggccatgacgtcgagcacggcgttcgcgacattgctcgcgacggcgtggccacccgtcgtgtgcccatagcgaaggccctgggcgatgggctcccggatgaacgtctccttgatcgacgaggtgaccgtcaccgcggccagcgggaggtacccgccgctgattcccttgctcatggtgacgatgtccggcgtgatcccgtcatggtcgaagccgaacatccggccggtgcggccgaatccgcagaacacctcgtcgaggatgagcaacgctccgtgctggtcgcacagttgccgcagcctggcgaggaatccggccggaagcacgacgcagccgccgagtcccagcagcggctcgaccatgaccgccgcggcgggcgggccggtttcaagtgccttggcgaacagtgcgatcagcgcatcggcgctttcctcggtccgcatcgcgcacggcgcggcgggcagggcgatgtgctcgatcgggaagggcggggcccattcgctggcggtgaacggcaaccccgagagctgctgagccaggtaggtcgtgccgtggtacgccgcctcgaaggtgatgacccggttgcggtcctcaccgatgttgcgccagtactgcagcgcgatcctgagagctgcttcggtggcctctgagccactgttgagcaggcaggtctcgttcagctcgcccggcaggagctcggccagccgcgatgccagcgtttcagcgggatcgtggctcgacaccatggggtcgtagtggacgagctgctcgaactgtcgactcgcagcttcgatcagccgcggatgtccgtggccgcaggacgcgttcaggacaccggagatggcgtccaggtaccacttgccctccgcgtcgcggacgcgattgccccgtgcctcgacgatccgcagcgagccggcctgctgggtgatcggcgtccaaggtcgccacagtgaactcgttgaagtggaactgtgcatgtcttaactctccaggggaccagtcgtcgggtcttcaggatttccgctcgggaaagctcgagattgccgtggtgagccagtggcgccagcgggtgccgaattcctgggctccgtagccggcgatctcctcgtcgaggaggagccggagttgaagttccgcgtcgcggacctgtacggcggccatgaacgagcacacctcaggggggcggctgtgagtcgacgtgacttcgacgcacggaacccccgcgatgtgcaccgtgcgctccgcagcgtgtgtgtagctgagcagcgccgtgaccgagccggagaacgtggatccgagagcggtgaccgcggggaacggcacgtccgcgtggtcgatctcccggtaccaactcctgacgaagtcacccgcggcgtccggtgtctggtgcgccccgggcaggtcgagcgagatgacggtgttcatgaaacacccgacaacgtcggcgtacgcggcgttccgcccgccccacgggtagccgatgacgctcggccccggctccgcgacgtctcgcagtgcgcgatggatcgagaagagaacgtaggggaacagggacccgcgaaaggagcgcgggacggcgacgcccgggagcgtatcgatgggaatgacgcgggtgtccttccccgtcgcccgggggaattcaccggcggcttccaggcggtccgcccagaatttgactccggggccgctcgcggccgcgtcctcgaatgctttccggtcatggatggcggcttgataacgtgccggctggctgtcgtccggggccgacggggcagccagctgccgtttgatgagcagcatcgactgttcgtcgaccaatgcgtgatcgagaaccagcagcaggttgtcgctctcgggtgagcgtatgagacgggccgccagcggcgcaccgtccagcgaggtttcgaattcctcgatcacctccgtcacacactccgacacggaatccccgcccgctgcgtggagttcggcgaaatcgcattcgtccggataccactcctggtaagcggtgccgcgggagaaccggatccggtaggacagcgcagggtttcggagcaccacggattgcaggacctgacgcacatctgccgtcgacaggcgggccggcgatgcacggaacatcaaggtgacggtccctctccgacccgcgcgctgcgcgtccaggccgaaggtcagttgtgcgctcaacaagggaagcctgtcggtcatagcggacctctatggcttgacggaccaccagcgacgctaccacccgatgtcaggggcgtcaaactgatcacctgtaggctggagctgcttcgaagttcctatactttctagagaataggaacttcgaactgcaggtcgacggatccccggaataattgcccacttgacgttgagagtgaagcaatataggttaacctgccacgtgttcgttatgagaggtggtcctcattgaacccatcctgctacgttggcgccgtgactgaagtagcgagggatttgcaggatgtagagtcgaagactgatggtccgagcctatggcgacagcgggatttcctcctgctgtggagtggtcagacggtcagtgagattggatcggctgtcacacgggtggctttgccgctggtcgcggtcgtctcgctccacgcgagcacgtttcaggtcgggttgctgaccgccgcaaccactctggcgttcgcggtgatcgcgctgcccgccggcgcgatcgtggaccgccgccccaagcgctccatcatgattgtctgtgatctgctgcgcctgctgatcctcggctcgatcccggtggcgggcgcgttcgacgtcctgacgatgggtcagctctacctggtcgcgatcgcggccggtgtgtgcaccgtgttcttcgacgtcgcttaccagagctacctgccctccctggtccgcaccgaggacctgatggccgccaacggcaagctcggcaccacccaggcgttcgcgcagctcggcggaccgagcctgggcggcggcctggtcgggctggtgggcgccgccggggcggtgatcgcggacgcgctgtcgtacgccgtctcgatgctggcgatcctcggcatccggcggcgggaggagccgccgccgccaccaccggccgacgagccgctgcgccgccggatcaccgagggcctgcgcttcgtcttcggacacccgatcctgcggcgggtcgtgatctgcaccggcgccgggaacctgttctccggcatgacctcggcgctggccatggtgttcctgatccgcgtcctgcatgtgagtcccgcgctgaccggcctgatcatggcgggctcagcgatcggcgcgatcgccggcgggttgttcgccgggcagctcgccaagaagatcggctcggcgcgcatcatctggatgtcgatgctggtcttcagcgcaccgcaggtcatcgcggcggccgcctggcagggctggggagtgctgctgttcccgctgggctggggcatcacgggcttcgccttcatggtctacaacgtcgcccaggtcagctaccggcagtcggtcaccccgcccgagctgatgggccggatgaacgcggccgtccgctgggtcgtgtggggcacgctgccgctcggcagcatcctcggcggcgcactgggcaccctgatcggcgtacgccccgccctcgtggtggccttcatcggctcctgggcggccggctggttcgtgttcttctccccgctccgccacctgcgcgacatcccccagaccgccacggattgacggtgagcacgggaccgctcgtggccacgcccggcgctgagcctccgtcatcgacaggagtcgtcgaccggccggcggcgcggttctgacgagcgcgcccgctgctttcagagcgagcaggacccacctctgccacccctgactccgctccggagaagggctcgtggccgagggcctggaagtcgggacggcgccggcgacttcggcgactgcctggagctcatcggcactcgctggttggacactagatcatgagggctgatacatggccatgggcttcaccgcgggcatcgcggacttcgaccagaagcagttcgacgcgctcgacgtacgggccggcgcggcctcctcctacggtcggctccgccagcacgaggaggaccgccggtgggccgcccgctacctcggatgggttgagggcgaggtgctgagggcggtcgtgccggtgtaccggcaccgcatgcggtcgtgggccgacccgtcgtacgacccccgcgcctggggtcttccggagggcgtgtccgacgagttcacgccggctacctcgcttctggtcggcggatgcctcgaccggcgcaccggtttccacgtcgaggcgggagccaggacgccgggcgagctgcggaggattctcgtcgagcttgcccggctcgccgccgacgaggaccgcggcctggtgttcccctacctgtacgacgacgcccgggacgcgctggcggcggcgacggaagaccgcgtcgtgtgggccgagctcgggcgggaggcccatctgtacggggtggccgatccgacgtgggagcaggtactcccgtccagggtgcgctaccggctccggcgggaccggcgcgtgatcgaggacgtccccatgacggtggctgaggagtcctgggacgatgtcgacgagtgggcttccccgttgatcgccgaccacaacgcggccaaggggcagcgggagccggccgagttcgtgagttttcgcttctcccgctggcaggagaacccggacgttcggctgctggccttcacggccgagtcggccggactgcggggcgttcagtcggtcctggtgtggggcgacgagctggaattgtacgagatcgggctggccggcgaggagagtgacgagcgcttggcgctgtacctcaacctgctcttccaccagccgatccggtacgcgcgaagcctcggcatcgatcacatacgtctcggctcgaaagcggagacggcgaagggacggcggggcggcgtcttcgccaccctgcacggcggagttctcggccgtgccgagacacgcgccctcgcgcgcgccggctcatgagagggaggcggctggtacccgccggcagccaccgggaagcggccgcacggcgggaggccatcacttcacgaaggctgtgccctcgaacgcttgaggtcggggagcagaccgaggtgttcctcccgcaccaggtcgaaccggagcgagaacgcgaccagggcctcgcgcttggagtgcatgcggccttcgtccacgtacttggcccactgactgaccggaagcttctgatccgtcaggtagtcgatgtggtagttgatgctgctgcggttcgcacccctgaactgcttgatccccttcagcctctcgaccacctcctgaacggagggcacggctgccatggaggaaccgcgcagacgcggctcgcacagtgcgacgagaacggcgaagtacttgctctccgggtccaacttggtcatcgcggactcagccaccgtggcggcctggtcaggtccgagcaggcgcggcggaggagtgaagacggtgagttcgctgatgctcgcgccggatgggatcaggacgcgcgacatctcgaacgggatcaccatgcccagctggcgggggcgcgccttgaccagctccgtgccgccctccaagttctcgatgacgaaggtggtactggtggtgaaattcgagaagaggaggtgatggtcggaaacctcgaacgcgccgatgctcggcgtagcgccgggctggaattctccggtgtagctggatatgccgaagttcagtcgatcgccgaccttcaggttgatccgttccttggcgacgggtccaccaggatggcgggtcttgttccgccaggtcacgatcacttctacatcggcttcgatcttggtgtgcatgaagagcgtcttcctgtcttcctcgaccacttgtgggggtttcaaggcggacccggtgccgatcagcatgtccgttgacactgcaggaggaaaagtggagatggagcgcttcaggaggatctggatgccctcctgcggattcacgtccggcgagtagccgggaagtaccggatctccagccagcctttttgcctcgctgcgaaatcggtcgcctccctcgaccgtccatttcacccgcggcgcacgagcgcgcggtcgaccacacgcgccccatgggcgggctcgatcccgcctcgtcccggctccggatgcgcggccacccaccgctcaccacgtgcacactgcacgccgagacgatcttgaaacgccggcgtttgctgactgctacgcacattcgtcccgagcagtcgacgcgacagcgtcactgagaaatccctgacgggatcaccggctgcggcgatctatcaggctgtcctgaacaggacgtgtcagatggctgaaatcgcggctggtcgactgggcgatccggcggcgaggtccaacgcctcgctgcggccacgctcatcgagcgtgccttcgtcccggacggcgaccacagcgcgggcggcgaccatcgggtcagagatggcgaccgctggctgaagaggtttctctgcgctcttcatcttaattcttcaccccgtggattcattgccaaagggcaccattccggcaacctctggcggtcaatcgatgcgcctacgcacggcgcccagatgcgtcgaccgaatggatttcatcggagaaatcctggtcgatttgcgcattttggaaaaattcaaaaaaataggcattgcacccttgaaggggcattcgcaacgtagtggacaactcccgtcatccgcacgtcatcgcagctcacccccttgagcaaaaggtgcccagcaggacaccgccagaccggcccatcacgtcgatcatgccgaaggccagttcgatcgggcgaatttccctctgtctcgatactggacgcgatgggcgatgtcggttatccatccatggtcaggtcggtgcacatccgcgggcaagggcggttttcagtcattcgactgatcgagccttttcaacgttgtcgctccagagtgagggcgaccgcggcgattgaccccattcgattgcgtgctctacgcgaagccgatcccgactacttcctgctggccggaatcccctgttcgcgcgctcggcgagcagcttgatgacggccgtcgcgtaggcgtgggcaacgcatgacagaggtacccaagccggccgcgatcggggcgacggagacacgtcggcgcaggtacaccggccaaaccggcgcacgctggcgcggcaggagcttccagcaccgggccccctccgaggcgacgacgcgcccccactcgaccagcgcgtgaggcaggtcgagtgcggcagggcggaaggccaacaaggctcctgtgcccgcgagttgagacgtcgagcatctttttcaacggcaggtgagatttgtccgttgtggacatcgatccctcgcccgatccctatagtgagtcgtattatgcggccgcgaattctcatgtttgaccgcttatcatcgataagctctgctttttgttgacttccattgttcattccacggacaaaaacagagaaaggaaacgacagaggccaaaaagctcgctttcagcacctgtcgtttcctttcttttcagagggtattttaaataaaaacattaagttatgacgaagaagaacggaaacgccttaaaccggaaaattttcataaatagcgaaaacccgcgaggtcgccgccccgtaacaaggcggatcgccggaaaggacccgcaaatgataataattatcaattgcatactatcgacggcactgctgccagataacaccaccggggaaacattccatcatgatggccgtgcggacataggaagccagttcatccatcgctttcttgtctgctgccatttgctttgtgacatccagcgccgcacattcagcagcgtttttcagcgcgttttcgatcaacgtttcaatgttggtatcaacaccaggtttaactttgaacttatcggcactgacggttaccttgttctgcgctggctcatcacgcaggataccaaggctgatgttgtagatattggtcaccggctgagggttttcgattgccgctgcgtggatagcaccatttgcgatcaggcgtccttgatgaatgacactccattgcgaataagttcgaaggagacggtgtcacgaatgcgctggtccagctcggtcgattgccttttgtgcagcagaggtatcaatctcaacgccaaggctcatcgaagcgcaatattgctgctcaccaaaacgcgtattgaccaggtgttcaacggcaaatttctgcccttctgatgtcagaaaggcaaagtgattttctttctggtattcagttgctgtgtgtcggtttcagcaaaaccaagctcgcgcaattcggctgtgcagatttagaaggcagatcaccagacagcaacggccaacggaaaacagcgcatacagaacatccgtcgccgcgccgacaacgtgataatttttatgacccatgatttatttccttttagacgtgagcctgtcgcacagcaaagccgccgaaagttcctcgaccgatgcccttgagagccttcaacccagtcagctccttccggtgggcgcggggcatgactatcgtcgccgcacttatgactgtcttctttatcatgcaactcgtaggacaggtgccggcagcgctctgggtcattttcggcgaggaccgctttcgctggagcgcgacgatgatcggcctgtcgcttgcggtattcggaatcttgcacgccctcgctcaagccttcgtcactggtcccgccaccaaacgtttcggcgagaagcaggccattatcgccggcatggcggccgacgcgctgggctacgtcttgctggcgttcgcgacgcgaggctggatggccttccccattatgattcttctcgcttccggcggcatcgggatgcccgcgttgcaggccatgctgtccaggcaggtagatgacgaccatcagggacagcttcaaggatcgctcgcggctcttaccagcctaacttcgatcattggaccgctgatcgtcacggcgatttatgccgcctcggcgagcacatggaacgggttggcatggattgtaggcgccgccctataccttgtctgcctccccgcgttgcgtcgcggtgcatggagccgggccacctcgacctgaatggaagccggcggcacctcgctaacggattcaccactccaagaattggagccaatcaattcttgcggagaactgtgaatgcgcaaaccaacccttggcagaacatatccatcgcgtccgccatctccagcagccgcacgcggcgcatctcgggcagcgttgggtcctgcagatccggctgtggaatgtgtgtcagttagggtgtggaaagtccccaggctccccagcaggcagaagtatgcaaagcatgcatctcaattagtcagcaaccaggtgtggaaagtccccaggctccccagcaggcagaagtatgcaaagcatgcatctcaattagtcagcaaccatagtcccgcccctaactccgcccatcccgcccctaactccgcccagttccgcccattctccgccccatggctgactaattttttttatttatgcagaggccgaggccgcctcggcctctgagctattccagaagtagtgaggaggcttttttggaggcctaggcttttgcaaaaagcttcacgctgccgcaagcactcagggcgcaagggctgctaaaggaagcggaacacgtagaaagccagtccgcagaaacggtgctgaccccggatgaatgtcagctactgggctatctggacaagggaaaacgcaagcgcaaagagaaagcaggtagcttgcagtgggcttacatggcgatagctagactgggcggttttatggacagcaagcgaaccggaattgccagctggggcgccctctggtaaggttgggaagccctgcaaagtaaactggatggctttcttgccgccaaggatctgatggcgcaggggatcaagatctgatcaagagacaggatgaggatcgtttcgcatgattgaacaagatggattgcacgcaggttctccggccgcttgggtggagaggctattcggctatgactgggcacaacagacaatcggctgctctgatgccgccgtgttccggctgtcagcgcaggggcgcccggttctttttgtcaagaccgacctgtccggtgccctgaatgaactgcaggacgaggcagcgcggctatcgtggctggccacgacgggcgttccttgcgcagctgtgctcgacgttgtcactgaagcgggaagggactggctgctattgggcgaagtgccggggcaggatctcctgtcatctcaccttgctcctgccgagaaagtatccatcatggctgatgcaatgcggcggctgcatacgcttgatccggctacctgcccattcgaccaccaagcgaaacatcgcatcgagcgagcacgtactcggatggaagccggtcttgtcgatcaggatgatctggacgaagagcatcaggggctcgcgccagccgaactgttcgccaggctcaaggcgcgcatgcccgacggcgaggatctcgtcgtgacccatggcgatgcctgcttgccgaatatcatggtggaaaatggccgcttttctggattcatcgactgtggccggctgggtgtggcggaccgctatcaggacatagcgttggctacccgtgatattgctgaagagcttggcggcgaatgggctgaccgcttcctcgtgctttacggtatcgccgctcccgattcgcagcgcatcgccttctatcgccttcttgacgagttcttctgagcgggactctggggttcgaaatgaccgaccaagcgacgcccaacctgccatcacgagatttcgattccaccgccgccttctatgaaaggttgggcttcggaatcgttttccgggacgccggctggatgatcctccagcgcggggatctcatgctggagttcttcgcccaccccgggctcgatcccctcgcgagttggttcagctgctgcctgaggctggacgacctcgcggagttctaccggcagtgcaaatccgtcggcatccaggaaaccagcagcggctatccgcgcatccatgcccccgaactgcaggagtggggaggcacgatggccgctttggtccggatctttgtgaaggaaccttacttctgtggtgtgacataattggacaaactacctacagagatttaaagctctaaggtaaatataaaatttttaagtgtataatgtgttaaactactgattctaattgtttgtgtattttagattccaacctatggaactgatgaatgggagcagtggtggaatgcctttaatgaggaaaacctgttttgctcagaagaaatgccatctagtgatgatgaggctactgctgactctcaacattctactcctccaaaaaagaagagaaaggtagaagaccccaaggactttccttcagaattgctaagttttttgagtcatgctgtgtttagtaatagaactcttgcttgctttgctatttacaccacaaaggaaaaagctgcactgctatacaagaaaattatggaaaaatattctgtaacctttataagtaggcataacagttataatcataacatactgttttttcttactccacacaggcatagagtgtctgctattaataactatgctcaaaaattgtgtacctttagctttttaatttgtaaaggggttaataaggaatatttgatgtatagtgccttgactagagatcataatcagccataccacatttgtagaggttttacttgctttaaaaaacctcccacacctccccctgaacctgaaacataaaatgaatgcaattgttgttgttaacttgtttattgcagcttataatggttacaaataaagcaatagcatcacaaatttcacaaataaagcatttttttcactgcattctagttgtggtttgtccaaactcatcaatgtatcttatcatgtctggatctgacgggtgcgcatgatcgtgctcctgtcgttgaggacccggctaggctggcggggttgccttactggttagcagaatgaatcaccgatacgcgagcgaacgtgaagcgactgctgctgcaaaacgtctgcgacctgagcaacaacatgaatggtcttcggtttccgtgtttcgtaaagtctggaaacgcggaagtcagcgctcttccgcttcctcgctcactgactcgctgcgctcggtcgttcggctgcggcgagcggtatcagctcactcaaaggcggtaatacggttatccacagaatcaggggataacgcaggaaagaacatgtgagcaaaaggccagcaaaaggccagcaaaaggccaggaaccgtaaaaaggccgcgttgctggcgtttttccataggctccgcccccctgacgagcatcacaaaaatcgacgctcaagtcagaggtggcgaaacccgacaggactataaagataccaggcgtttccccctggaagctccctcgtgcgctctcctgttccgaccctgccgcttaccggatacctgtccgcctttctcccttcgggaagcgtggcgctttctcatagctcacgctgtaggtatctcagttcggtgtaggtcgttcgctccaagctgggctgtgtgcacgaaccccccgttcagcccgaccgctgcgccttatccggtaactatcgtcttgagtccaacccggtaagacacgacttatcgccactggcagcagccactggtaacaggattagcagagcgaggtatgtaggcggtgctacagagttcttgaagtggtggcctaactacggctacactagaaggacagtatttggtatctgcgctctgctgaagccagttaccttcggaaaaagagttggtagctcttgatccggcaaacaaaccaccgctggtagcggtggtttttttgtttgcaagcagcagattacgcgcagaaaaaaaggatctcaagaagatcctttgatcttttctacggggtctgacgctcagtggaacgaaaactcacgttaagggattttggtcatgagattatcaaaaaggatcttcacctagatccttttaaattaaaaatgaagttttaaatcaatctaaagtatatatgagtaaacttggtctgacagttaccaatgcttaatcagtgaggcacctatctcagcgatctgtctatttcgttcatccatagttgcctgactccccgtcgtgtagataactacgatacgggagggcttaccatctggccccagtgctgcaatgataccgcgagacccacgctcaccggctccagatttatcagcaataaaccagccagccggaagggccgagcgcagaagtggtcctgcaactttatccgcctccatccagtctattaattgttgccgggaagctagagtaagtagttcgccagttaatagtttgcgcaacgttgttgccattgctgcaggcatcgtggtgtcacgctcgtcgtttggtatggcttcattcagctccggttcccaacgatcaaggcgagttacatgatcccccatgttgtgcaaaaaagcggttagctccttcggtcctccgatcgcccttcccaacagttgcgcagcctgaatggcgaatggcgcctgatgcggtattttctccttacgcatctgtgcggtatttcacaccgcataaattccccaatgtcaagcacttccggaatcgggagcgcggccgatgcaaagtgccgataaacataacgatctttgtagaaaccatcggcgcagctatttacccgcaggacatatccacgccctcctacatcgaagctgaaagcacgagattcttcgccctccgagagctgcatcaggtcggagacgctgtcgaacttttcgatcagaaacttctcgacagacgtagatcaggcttcccgggtgtctcgctacgccgctacgtcttccgtgccgtcctgggcgtcgtcttcgtcgtcgtcggtcggcggcttcgcccacgtgatcgaagcgcgcttctcgatgggcgttccctgccccctgcccgtagtcgacttcgtgacaacgatcttgtctacgaagagcccgacgaacacgcgcttgtcgtctactgacgcgcgcccccaccacgacttagggccggtcgggtcagcgtcggcgtcttcggggaaccattggtcaaggggaagcttcggggcttcggcggcttcaagttcggcaagccgctcttccgccccttgctgccggagcgtcagcgctgcctgttgcttccggaagtgcttcctgccaacgggtccgtcgtacgcgcctgccgcgcggtcttcgtacagctcttcaagggcgttcagggcgtcggcgcgctccgcaacaaggttcgcccgttcgccgctcttctcaggcgcctcagtgagcttgccgaagcgtcgggcggcttcccacagaagcgccaacgtctcttcgtcgccttcggcgtgcctgatcttgttgaagatgcgttccgcaacgaacttgtcgagtgccgccatgctgacgttgcacgtgccttcgtgctgcccaggtgcggacgggtcgaccaccttccggcgacggcagcggtaagagtccttgatcgattcttccccgcgcttcgaagtcatgacggcgccacactcgcagtacagcttgtccatggcggacagaatggcttgcccccgggaaagccccttgccgcgccccctgccgtccaaccacgcctgaagctcataccactcagcgggctcgatgatcggtccgcaatcaagctcgaccggccggagcgtgatcgggtcgcgctgaatgcggtaaccctcaatcttcgtggtcggcgtgccgtccggcttcttcttgtagatcacctcagcggcgaagcccgcaatacgcgggtcccgaaggattcgcataacggttgccgggtcccaggcgcttgaagcggtcttcttcccaatcgtctcgccccgggtcggcacggcgtcagcgtccatgcgcttacaaagccccgtgatgctgcccgggtgaatggcggcttgactgcccggcttgaagggaaggtgtttgtgcgtcttgatctcacgccaccaccaccggattacgtcgggctcgaactcgaagggtccggtaaggggagtggtcgagtgcgcaagcttgttgatgacgacattgaccattcggccgttgcgcgtgatctccttcgtctccgaaacaagctcgaagccgtaaggcgccttcccgccgacgtacccgcccaattcgcgctgaaggttcttcgtgtcgagaatcttcgccgacttcagcgaagattctttgtgcgacgcgtcgagccgcataatcaggtgaatcaggtccatgacgtttccctgccggaagacgccttcctgagtggaaacaatcgtcacgcccagggcgagcaattccgagacaatcggaatcgcgtccatgaccttcaggcgcgagaagcgcgacacgtcatagacaatgatcatgttgagccgcccggcgcggcattcgttcaggatgcgttcgaactccgggcgctccgccgtcccgaacgccgacgtgcccggcgcttcgctgaaatgcccgacgaacctgaaccggcccccgtcgcgctcgacttcgcgctgaaggtcggccgccttgtcttcgttggcgctacgctgtgtcgctgggcttgctgcgctcgaatttcgcgctcgcgcgactgacggtcgtaagcacccgcgtacgtgtccaccccggtcacaaccccttgtgtcatgtcggcgaccctacgcccccaactgagagaactcaaaggttaccccagttggggcactactcccgaaaaccgcttctgacctgggaaaacgtgaagccccggggcatccgctgagggttgccgccggggcttcggtgtgtccgtcagtacgggccatagaggggcgtcgtgtaacccacccagggcgattgctccggcacggggaagccgcgccacgccttcgggacgtctcaggtcgaggtggcccggctccatgcaccgcgacgcaacgcggggaggcagacaaggtatagggcggcgcctacaatccatgccaacccgttccatgtgctcgccgaggcggcataaatcgccgtgacgatcagcggtccagtgatcgaagttaggctggtaagagccgcgagcgatccttgaagctgtccctgatggtcgtcatctacctgcctggacagcatggcctgcaacgcgggcatcccgatgccgccggaagcgagaagaatcataatggggaaggccatccagcctcgcgtcgcgaacgccagcaagacgtagcccagcgcgtcggccgccatgccggcgataatggcctgcttctcgccgaaacgtttggtggcgggaccagtgacgaaggcttgagcgagggcgtgcaagattccgaataccgcaagcgacaggccgatcatcgtcgcgctccagcgaaagcggtcctcgccgaaaatgacccagagcgctgccggcacctgtcctacgagttgcatgataaagaagacagtcataagtgcggcgacgatagtcatgccccgcgcccaccggaaggagctgactgggttgaaggctctcaagggcatcggtcgacgctctcccttatgcgactcctgcattaggaagcagcccagtagtaggttgaggccgttgagcaccgccgccgcaaggaatggtgcatgcaaggagatggcgcccaacagtcccccggccacggggcctgccaccatacccacgccgaaacaagcgctcatgagcccgaagtggcgagcccgatcttccccatcggtgatgtcggcgatataggcgccagcaaccgcacctgtggcgccggtgatgccggccacgatgcgtccggcgtagaggatccacaggacgggtgtggtcgccatgatcgcgtagtcgatagtggctccaagtagcgaagcgagcaggactgggcggcggccaaagcggtcggacagtgctccgagaacgggtgcgcatagaaattgcatcaacgcatatagcgctagcagcacgccatagtgactggcgatgctgtcggaatggacgatatcccgcaagaggcccggcagtaccggcataaccaagcctatgcctacagcatccagggtgacggtgccgaggatgacgatgagcgcattgttagatttcatgacattgcactccaccgctgatgacatcagtcgatcatagcacgatcaacggcactgttgcaaatagtcggtggtgataaacttatcatccccttttgctgatggagctgcacatgaacccattcaagacgtcatggcaatcgctagagcttgcatgcctgcaggtcgacggatcttttccgctgcataaccctgcttcggggtcattatagcgattttttcggtatatccatcctttttcgcacgatatacaggattttgccaaagggttcgtgtagactttccttggtgtatccaacggcgtcagccgggcaggataggtgaagtaggcccacccgcgagcgggtgttccttcttcactgtcccttattcgcacctggcggtgctcaacgggaatcctgctctgcgaggctggccggctaccgccggcgtaacagatgagggcaagcggatggctgatgaaaccaagccaaccaggaagggcagcccacctatcaaggtgtactgccttccagacgaacgaagagcgattgaggaaaaggcggcggcggccggcatgagcctgtcggcctacctgctggccgtcggccagggctacaaaatcacgggcgtcgtggactatgagcacgtccgcgagctggcccgcatcaatggcgacctgggccgcctgggcggcctgctgaaactctggctcaccgacgacccgcgcacggcgcggttcggtgatgccacgatcctcgccctgctggcgaagatcgaagagaagcaggacgagcttggcaaggtcatgatgggcgtggtccgcccgagggcagagccatgacttttttagccgctaaaacggccggggggtgcgcgtgattgccaagcacgtccccatgcgctccatcaagaagagcgacttcgcgaagctggtgaagtacatcaccgacgagcaaggcaagaccgatccccggggacctgcaggtcgactctagctagctggactcaaccaagtcattctgagaatagtgtatgcggcgaccgagttgctcttgcccggcgtcaacacgggataataccgcgccacatagcagaactttaaaagtgctcatcattggaaaacgttcttcggggcgaaaactctcaaggatcttaccgctgttgagatccagttcgatgtaacccactcgtgcacccaactgatcttcagcatcttttactttcaccagcgtttctgggtgagcaaaaacaggaaggcaaaatgccgcaaaaaagggaataagggcgacacggaaatgttgaatactcatactcttcctttttcaatattattgaagcatttatcagggttattgtctcatgagcggatacatatttgaatgtatttagaaaaataaacaaataggggttccgcgcacatttccccgaaaagtgccacctgacgtctaagaaaccattattatcatgacattaacctataaaaataggcgtatcacgaggccctttcgtcttcaa

SEQ ID NO: 2 - DNA, 48636 bp, synthetic construct
  misc_feature 1..48636: note = Cosmid pIJ787 containing modified napsamycin gene cluster from Streptomyces sp. DSM 5940
  source 1..48636: mol_type = other DNA
atcggtacctcgacgaggttcatcgcgggggagccgatgaagccggcgacgaagaggttcgccgggcggtcgtacatgttgcgcggcgagtcgacctgctggagcagcccgtccttcagcacggcgacccggtcacccatggtgagggcctcgacctggtcgtgggtgacgtacacggtggtgatgccgagacggcgctgcagcgaggcgatctgcgtacgggtggagacacggagcttggcgtcgaggttcgacagcggctcgtccatgaggaagacctgcggctcccgcacgatggcccggcccatcgccacacgctgacgctgaccaccggagagcgccttcggcttgcggtccaggtactcggtgaggtccagcatcttggcggcctcttcgaccttcgcccggatctcggtcttgttcacaccggcgatcttgagcgcgaagcccatgttgtccgcgacggtcatgtgcgggtacagcgcgtagttctggaacaccatggcgatgtcccggtccttcggcggcaggtgcgtgacatcgcggtcaccgatacggatcgcgccgccgttgacgtcctcaagacccgcgagcatgcgcagggaggtcgacttgccacaaccggagggaccgacgaggacgaggaactcaccgtccgcgatgtcgatctcgagctggtccacggccggcttcgtggagccggggtagacgcgggacgccttgtcgaacgtgacactggccatgatggatcttctcctcaaccggcaggaacgtgccggacgatccgagtagggagtggtctggtccactgagtggacctgcggtgacgctacctggcgttccccgatctgtcagtagtccggagcacacggaaatcgcggacgccggaggtccggcgttggttagactgctccggcacgcctccttagctcagctggccagagcaacgcacttgtaatgcgtaggtcgtcggttcgaatccgacagggggccctctgggaagcccaggtcaggaccatgacctgggcttccgtgtgccatcggtcttttggatcgggcccatcgaccccatcggacaccggcgacccatggatggtcgtatgtccagccgtgaacccttggcagatggaccccgtgccgtgggactgccggtggacagccgcgcgtgacggcccgccttccggagtccggtgtgagccgcgggtgactcggggcctgcaaggccggtcagcgtccggaaaccgctcttccgcagccccgcaaccgcccactcggggcggcggcctctccgaagttcctgacggatgtcagtacaggtcagcgcaccgggcggcatgtactgaacgaggatggggacgtgctgtcgtcccctgacccgccttcgcacggatgaaccgacgtcccgccgtgccgaggccgggaggccggtccgcggacacccatcgagaaagggcgacaccatgtcggaccaggatcgtcgggcacggttgatccgtgccctggagtaccggcagatcttcgacgaccggctcgaccggatcgagcggcaggttccgttcgactcggtccacgatgtcgacacctcggaatccgtggagctgtgggaactcccccagggcgaccagctccaggtgggacgggacgcgcggtactcacccacaccggtccgcacggtgcgccacgtgctcggccagtgcgacgtgaaacacgaggacatgacgttcgtcgacgtcggctgcggcaaggggcgggtccttctgcaggccaccgagttccctttccggcgcattgtcggtgtcgaggcgtcagagacgctctgcgacatcgcccgggccaacgtcgagaaggcgtcggcgacactcgagggctgcgaccggatcgatgtggtgcacgcagacgccacccggttcgacgtcccggacgacgccgggctcttctacttctacgagccgttctccacggaagtgtcctcggccgtactggagaggatcgaggattccgtgcgccgtcacccgcgtcccgtcgtcctctgcttcaccggccggggccagcccgacggccaggccggcgagcacgacacccctccagttgccgccgccgccgcggagattcgaccccgatggaagcggatcggcaccgtcagctccccggacgccgtgttctacgactccctgctgtacgcgtacgaggaccacggctcgttcgaggcccaggccgtcccggattcctgagaggcaaaccatgcgcgctgccatgaccgccgcagagcagcggtctctgctcgacacggccgtttccctgcccgatctcttccgcgctgttgctgcggcccgtggtgccgccccggccctccgagacggcgagcggaccctcagctaccgcgagctcgacgacctgacggaccggatcgccgcacgcctggcggcggaaggggtccgaccgggcgaccgggtggggatcctcctcccacgctcggccgagacgcagatctccatcctggccgtcctcaaggccggagccgcctatgtcccgctcgacccctcctatccggcggagcggttgcgcttcctggtacgcgacgctgacatcggggtggtcgtcggcgacgccgggcactgcgctgccggcgggctcaaggatgtccgtgtcctcgcccccgaggccgaggagacgatcccgccggcgccgcccgtccccctcgacggcagcgaattggcgtacgtgatctacacctccggctcgaccggcacgcccaaggggtgcatggtccagcacaccagcgtcctcgacctggtccgcggcgtgatgtcggtggtcgacctggacacggaggaccgcgtcgggctcttcctcccgttcatcttcgacgggtccgtcctccagttctggctctccctggcggccggcgcgacggccgtcgtcgtcccggcccgggtggcgcagtcgatgcccgacttcctcgacctgcttcgacgcgaggccgtgaccctcgtcatacaggtccccacgacgctgcgggcgctcgcccacgcccacgaggcggcgggccggcctcccctcgccctccggtacgtcctggtgggcggcgagagcgtggagcttgatgtcgtctccgccttcctcgcgcgctgcccgggcacgccgcccgaggtcgtcaacatctacggaccgaccgaggcggcctgcgtcgccacctgtcgcgtgctgacccaggaagacttcgacggccccgtgccctcaccgatcggtacggcgctgccgcacctgctcgtcgaggtacgcggcgaggccatggagccggtcccggacggagaggtcggcgaactggtgatagccggctcgggcgtggccgtgggctacctggggcgccccgaactgacagccgaacgcttcgtcgtcctcgacactccgcaggggccggtgcgctactaccggaccggggacctggccagacggctgccggacggcgccttcgcgtacctgggccgcaacgaccagcaggtcaaggtgcgtggcatccgtgtggaactcggcgaggtggagacgtatctgcgtgcccacccgatggtcagggaagccgccgccacggtggtcgacacccaggccggcgcccagttcctgaccgcgtgtgtggtgctcgccgaccaagcaccggaaaagcccgaggcgttgctgcggcagcacatgctcgcttcccttccgcccttcatggcgccggatcgctatcagttcgtccctgagctgccgtcgacggactcaggcaagctggaccgccgcgctgtgcacgacatggcaactccgcgtcgagctccccgcccctgatcgagtcgccggagccctcctggccggtgcgcggaagcgcgagaccgctgctgcctttcggcagcagcggtctcaggctttcgggggagtcccgtgctgaatcaattccggggatccgtcgacctgcagttcgaagttcctattctctagaaagtataggaacttcgaagcagctccagcctacagctcacgccgccccgtcccgtgtgaacggccagatgcacatacggacgatcgggactgggcagatgggtggcgcggccgaagggcggtcgtagaagggaacactcgtctgcagtgagcgagatgccctccaccctcccgaccaacgcggaaacgcgggatgcgcgtcgcttgatctcctctcgcgccgcacgggccagcgcaagctcgtgtccggaaaggtgccttctctgcgcggcgtcttcgagcagccgaactgattcagcagcgggcgcccggccgagctcccccatcgcttcggacgcatcggcaggaagtgcacgaggcagagggggggactcatgagttcgctgcacctgcgcagcctccttgaatgtcggtgtggacgggcccccgggccgccgccggaggcgttcagtcgagccaggtcagcaagtgacggagctcatcacgcagttgggcgacggtcggacgccgcacttcgatgtccgtcttcgtctgctcgccgaccggcgaggtccggtaaacgtgggtgaactcctccacggcgggcagctggaggaccagcgacgccgccgccttgcccgcggagcgggagatgcagtgcaggacctggtgatcgatgtgatagacggtccccgccggaaggagcgcttcgaacacggaagtcagtcgttccttgccctgcgccaccagggagaaggtctttccctgcccgatcggcaggtacttgtagtagtggtactccgtacccgggccgaccctgaactcctgcgcgaagtactccccgaccacgagcgcggtcgtgaagtcccagcggtgcgagtggatatcctcggtgatgctccctgtcgcgtccggctggggatgccacatgtggagacgcagccgccaggggttcttgtcgccggccagcagcacgagcttcaggaagttgttggcgtggtagtacgagcgggccgcgacgtcggcgagaacgtcttcgtcggcgatgatctggccgatcagagaacgcagttcggccggcgcggcgagccggcgaaccactgactccgagccctggaacgtcgtgccgtgcccgctgtccacgaccacttccaggtggtctttgacttcctgcagggacgcccctgccagagcctgcaccataacctgtacctccggtttcggacgctggcggttccagcgagtcgatggttggggtggggcgtaccgtgtgtcgacggccgcctttccggttctgttgactgcgggccggccagtccgggcgctagtcctcaccgagggcgaccaggaacgcgggggccccttcgaacggcgaccggccctgggccgtgatgatgttgtcagcgatcagcaggtcgccgcggcgccaccgcacgtgggtccgcaccgcgtcgtaggcgtgctggacggcggccaagtcatcgtcggacagcgtcgtcccgtcgccgaagtaggtgttcgtcggaaggtacttcccgaacgtctcggtcatgaccctgcgctcgacgggatccagattcccggcgttgaggaaggagatctggttgaaccagcactcctccccggtcgtcgggtgggcgaggaagccggggcggtggcgcatcgtgtgcagcgtgccttcggggagccacgaggactcgatcccggcggcccggagcacctcgtccagtgcggcgctgtccggaacggagaacgcctcctgccacgagatcccgaacttggcgtgaaaggaccggctcatcatccagccttcagcgcggacacggtcggcgagatgcgccggcaggtgctcggccatccggcgcatgtccccgaggtgggtccgccccgcgccgtccggcggtgcgaggcacgcggtgagcaccacggtggggaacgtcctgctgaaggatgcttcctggaacgggcagatcatacggtcgcccggccaggtgatcggcgagacgatgccgttcccgaagtcgctgcggttgttgaacgcctccgtgggggtgtgagcggcgatacccagggcgtcgcgcgcccggacgaggccctccggcccgtccagggggaggccgtggacgagtacggctccgtgggccaggcgctggtcccggatcgtggcagccgcttcccgcagccacgtgaacggttcgtcgccctcggcgtcgaagcagggcacgagcgcttccggcagcggagggacggtctgcctcacggggtctccttgtctccgatcggttcagcgtcgggccagggcgacgtcgacggcaccgctgatcttcgcgaccgcctccgccgtgtcgtcgtcggtcagcgtcagcgggggagcgatccggatcacgccgcgctccgcgcgcgtcatcacgcccgcccgcgccgaggcctcggcgatggcggcggctgactccggcgtgtcggcctcgatggcgaccaccaggccaagcccgcggacatcggtgatcagcgggttcgtcccgagcttccgcaggccctccagcagcgcgttcccctgggctgccgcgttctccacgagcttctcgtcggccatgacgtcgaggacggtgtttccgacggcgctcgcgacggcgtgtccgcccgtcgtgtgcccgtaccggagcccctgcgcgacgggttcccggacgaacgtctccttgatccgggaggtcaccgtcaccgccgccagcggtacgtagccgccgctgatccccttgctcagggtgacgaggtccggggtgatcccctcgtgctcgaacccgaacatccgtccggtgcgcccgaatccgcagaacacctcgtccaggatgagcagcgccccgtgccggtcgcacaactcccgcagtcgcgccaggaacccggccgggagcacgacgcagccgccgaggcccagcagcggctccaccatgaccgcggcggcgggcgggccggcttcgagcgcccgtgcgaacgcggcgatcagcgcgtcggcgccctcctcggtccgcagttcgcgcggtgccgccggcagggcgacgtgctcgatcgggaacggcggcgtccactcgctgacggtgaacggcagcttcgagagctgctgcgacaggaaggtcgtcccgtggtacgccgcctcgaaggtgatgacgcggtcacggtgctcgccgatgttccgccagtactggagcgcgatccgcagggccgcctccgttgcctctgagccactgttgagcaggaccgtctcgttcaggtcgcccggcagcagctcggccagccgggcggccagggtctcggcgggatcgtggctcgacaccatggggtcgtagtggacgagctgctggagctgccgcgtcgcggcttcgatcagccgagggtgtccgtgcccgcaggatgcgttgaggaccccggagatgccgtccaagtaccagttgccctccacgtcgcggacccggttgccgagcgcctccacgatgcgcagggagccggcctgttgggtgatcggtgtccagggccgccacagtgaactcgtccgagtggaagggtgcatttcgtgactctccaggtcgtcggttcttcagggtttcggttcggggacgtgtgagaacgcggaggtgagccggtcacgccagcgggtgccgaacgcgcggactccgtaggtggtgttctcctcgtcaagaaggagccggagccgcagttcgccgtcgtggagtgtcacgccggccagcagcccgcacatcgagggcggctcgctgcggctcggggtgacctcgacggccgggacaccggcgacgtcaacagtgggcggcccggcatgcgtgtagctgagcatggccgagaccgcgccggagaacgtggagccgagcgcggtgaccgcggtgaacggcacatccgcgtggtcgagctctcggtaccagttccgaagaaagtcgcccgtggggtccggagaccgagggcatccgggcgtgtccagggacacgacggtgttcatgaagcacccgacgacatccgtgtaggcggcgttccgcccgccccacggatagccgaccgtggtgggcgcgggctcagcgacgtcgcgcagggcgtggtggatcgagtgcaggacgtaggggaacagcgacccacgaaacccgtgcgggacggcgacgctcggaagggtttcgacgggaatggcccgagtggtccgggccgagggccgctggaattcgccggcggactccagacgttccgtccagaactttgtcccggggccgtcggccgcttccgtctcggatttcacccggtcgaaaacggcgttccgatatcgctccatccggtgctcgtcaggtgcggacggggcgcccagttgccgtttgatcaaacgcaccgaatgctcatcgaccaaggcatgatcgagaaccagtagcagatggtcgcccgtgggcgaccgaatgaggcacgccgtcatcgaggcgccgtccagcgaggcttcgaattcctcgacaacccgctccacggattccgcgaccgcttcctcgtccaacgcgcggagttcggtgacatgacactcggacgggttccactcctggtacgcggtgccccgggagaaccggatccggtgggacagtgcgggattgctgagcagcacggactccaggacctgacggacgtcctcggtcaccagtcgggccgacggcgtacggaacatcatggtcacggtccccctgcgacccgaacgctgcgcatccaggccgaaagccagttgggcactcgacaagggaagcctgtcgatcatgcggtccccctgatttcttacttggactgctgttctgcggcttacatccggcgctgcgagcagaatcggagaagatgactgaatattgccgaaaggttggcgagatctcttgcgatgccgactggtgaagccaacgcaacaccacgctcacgcccactgcgacgcgtcctcatattgcccgttcctcagccctcgggggtcctaacaggtaacagggctcagcggctcaactcctttatcgggccgtgctaggttgcccgccatgacggaagtggcgaacgattctcagggtgtcgaaacagaagtcgaacgcccgagtctttggcggcagcgcgacttcatgctcctgtggagtggtctgacgctcagcgaggtgggatcggcggtcacccgggtcgccctgccgctggtcgcggtcgtcgtcctcgacgcgagcacattccaggtcgggctgctcacggccgccaccaccgcggcgttcgcggtgttcgcgctgcccgccggcgcgatcgtggaccggcaccgcaagcgctccctcatgatcgtctgcgatctgctgcgcctgctgatccttggctcggtaccgctggccgccgccttcgacgtgctgacgatggggcagctctacatggtcgcgctcgcggccggtgtgtgcaccgtgttcttcgacgtctcgtaccagagctacctgccctcgctgatccgcaccgacgagctgatggcggccaacggcaagctcggcaccactcagtcgctggcgcagctcggcgggccgagtctgggcggcgggctggtcgctctggtgggcgctgccatggcgatcgtcgtggacgcgctgtcctacgctctctcgatgctggcgatgctcggcatccggcggagggaggagccgccgcccccgccgcccgcggacgagccgctgagccgccggatcaccgaggggctgcggttcgtcttcggccacccgatcctgcgccgggtggtgatctgcacgggcacagggaacctgttcggaggcatgaccgcggcgttggccatggtgttcctggtccgcgagctgcacgtcggcccggcgctgaccggcctgatcctggcggtttcggcgatcggcggcatcctcggggggatgttcgcgggcaggctcgccgagcgggtcggctcggcccggatcatctgggtgtccttgctggtcttcagcgcgcctcaggtcatcgcggcggctgcctgggagggctggggcgcactgctcttcccgctgggctgggcttgcgccggtttcgcgtacatggtctacaacatcgcccaggtgacctaccggcagtcggtgactccaccggagttgatgggccggatgaacgccgccgtccgctgggtggtgtggggcaccatgccgatcggcagcctgctcggcggagcgctcggcagcctgatcggagtgcgccccgccctcgtggtggccttcgcgggttcctgggcggccggctggttcgtgttcttctcaccgctccgccgcatgcgggacatcccccgacccgaagcgggttgagggcgccggaacgggacgactgcccggggcatcggatcgagaggactgacacatggccatgggcttcaccgcgggcatcgcggacttcgaccagaagcagttcgacgcgctcgacgtacgggccggcgcggcctcctcctacggtcggctccgccagcacgaggaggaccgccggtgggccgcccgctacctcggatgggttgagggcgaggtgctgagggcggtcgtgccggtgtaccggcaccgcatgcggtcgtgggccgacccgtcgtacgacccccgcgcctggggtcttccggagggcgtgtccgacgagttcacgccggctacctcgcttctggtcggcggatgcctcgaccggcgcaccggtttccacgtcgaggcgggagccaggacgccgggcgagctgcggaggattctcgtcgagcttgcccggctcgccgccgacgaggaccgcggcctggtgttcccctacctgtacgacgacgcccgggacgcgctggcggcggcgacggaagaccgcgtcgtgtgggccgagctcgggcgggaggcccatctgtacggggtggccgatccgacgtgggagcaggtactcccgtccagggtgcgctaccggctccggcgggaccggcgcgtgatcgaggacgtccccatgacggtggctgaggagtcctgggacgatgtcgacgagtgggcttccccgttgatcgccgaccacaacgcggccaaggggcagcgggagccggccgagttcgtgagttttcgcttctcccgctggcaggagaacccggacgttcggctgctggccttcacggccgagtcggccggactgcggggcgttcagtcggtcctggtgtggggcgacgagctggaattgtacgagatcgggctggccggcgaggagagtgacgagcgcttggcgctgtacctcaacctgctcttccaccagccgatccggtacgcgcgaagcctcggcatcgatcacatacgtctcggctcgaaagcggagacggcgaagggacggcggggcggcgtcttcgccaccctgcacggcggagttctcggccgtgccgagacacgcgccctcgcgcgcgccggctcatgagatcgcgcccgttgccaccttcgtggcttgccgtgcctcaagacatcgttgcgcgcgcaggagtttgacgtcggggaggagggcgaggtgttcctcgcggaccaggtcgaagcggagcgagaaggcgaccagggcctcgcgcttcgaatgcatgcgcccttcgttcaggtacttggcccactggctgaccggaagcttctggtcagccagatagtcgatgtggtagttgacgctgctgcggttggcgtccctgaactgctcgaccccccgcagtctttccaccacctcctggacggagggcacagccgccatcgaggaaccgcgcagacgcggctcgcacaaggcgacgagaacggcgaagtacttggtcgtcgcgtccagtttggacatcgcggactcggtgggcgtggcggccatctcgggcccgagcaggcggggcggggatgtgaagacggtgagttcgccgatgcttgcgctggaggggatgaggatgcgcgacatctcgaacgggatcaccatgccgagctggcgggggcgcgccttgacgagttcggtcccgccctccagattctcgatgacgaacgtggtgctggtggtgaagttcgagaagaagaggtgctggtcggacacctcaaaagtgccgatgctgggcgtcgcacggggctggaattctccgccggcgttgggtatgccgaagtccagccgatcgccgaccttcaggttgatcctttcctgggtagtggatccacccaggtggcgggcctggacgcgccaggtcagaatcacttctgcatcacgctcgaaaaggttgtccatggtgcccttcctgtcatcttcgacttcttgtgggagtgcaaaggaggagggttccggtcggctagggtgtggtgtgttccctaggtggaagcctgacgatgtgcagctgcagaaacgaatctgcacttacggtgaattgtttacccgcttgctcgtccattctcgaaggcattgctttcgatgggctctgccgatgctgaaattgttgaaatgttgatggcgtatcgctcatgcgccggtggtgcttgctctccgagaatggcttgaggaatccttgtcagtggatcctcgattcgaatggcgatccttgctccgcctcgctcggtctgtcaaggcctcccgtagggtctgactgatcagatcaagccaaggtgatcgcaatccatttacctctacatcttgacttgcgggcttggcaaggagttttcggtcttgggagattcgtggcgtcgaatccctattgcgtgtacgcgtccggacagcggtcggctcgacattgaggacgggctgtgtccgcaggtacgccgggcgcgagcccgcccggacgtgcgcgagcgacccgcgtatctggacagtctcctgacggatgtcagtacaggtcggcacgtccggcgtcatgtactgaatgagttaggggacgtggtgtcgcgttgggcttttttcccgatcgggagttaggggttggcggggtctatggctctcacgctggtcgagcgatttctgcgcggactggagatttcagccgaccgttccgcactgcgggtcggttcggaggacgtgacgtaccagcaggtgcacgacacggctctgatatgggcgggtgcactgcggaccaacggttctccgggcgcggtcggtgtgctgacggggaagagcgtaacgacttatgtggggcttctggcggtgctgtacgccggtggcacggtcgttccgcttcagccgagtttccctgccgcgttgacgcggcgcatgatgaagacggccggcgtgagggaggtcatcgcagatgagcgtggcctggcggtactgccggaggtcgtcagggatggtatgaccgtccgcgtcctcgacaacggcggttccgttacgggattcccgctgattcctgtatccgctgaatcggcgcttgccgaaccggtcgaggtggaactcgccgacccggcgtacattctcttcacgtcaggttcgacagggatccccaaggccgttcccatcgcacaccgcggtttcgcgcactatttcgacgagatggaccggcggctggacttcgggccggacgatgtgctgtcgcagaccttcgacctcaatttcgaccccggaatccacgacgtcttcgccgcgtggggtgcgggcgcgacgctccaggcggtgccgccgtccgcgtaccgggacctcccggggttcgtcgccgagcacgggatcaccgtctggcattccacgccgagcggcatctggatggcgcgggagatgggtgccctggaaaaaggcgccctcgacggtctgcggtggtccttcttcggcggggaggccctgcgctgccaggacgtgctggactggctggtggcggcgcccggatcgaaggtggagaacctctacgggccgacagagttctcgatcggcgtgtgctggcaccgctgggcgggcgaggagtcgcagcgccgcggggtgaacggcacggtcccgatcggcaaggtccacgcggtcaacgactttcgcctggtgaccgaggacggcgaacaatcctcggtggaaggcgagttgtggctcaccggaccgcagatctcgaccggctacctcgatccggccgagaacgaaggacggttcgtggtcgccgacggacggcgctggtaccgcaccggtgaccgggtccgggcacaaccggatggcgagctcgcctacctcgggcggatggactcgcaggtgaagattcacgcctggcgggtggagctcgcggaggtggaccacgtggtgcgcgcctgcgccggggtgctcgacgcggtcaccgtcacccggtcggccgcgcacggcgaggaactggtggtcttctacaccggcgacgaggtgcctgatcaggagctggccgacggtgtgggcgccgtgctcccggacaccgtcctgccgcggcagtacgtccacctggagagcctgccgctcaatcccaaccggaaggtcgaccgcctcgccctgaggaagcgggccgaggaactcgccggctgagccggacggcacacagacgtgaagtcgccacgaccgaactccgacggtgatcgcatgaagcccagcggacctgacgcccggcccacgtccctcggggacgggcctcccctcatggcgcctcgcgtcatgcccgcactgccaccgagaatcttttccgacgccgagtgggagcacatccgggcgggctgctcgcgcggcaggagcggtgcgaaatggaccgcccgctgccgtggagacgtgctccggctctaccggagcgagaccggttacggaatctacgaagccaccttcgtgccgaccgcggacggcgggcggcggatcgcacgtgcgctggtcgaggggcacccccagcggtaccggtccccgtccaccgagtacgacgccctcgtcctcgagctggtcgtcagcgcggtcctgctcgacgaaccagccgacggactccgcgccgcgatgacccgtctgatgcgtgccgcgtcgggcgttgtcgacatgccttccgaggtggtcgagcacagcatcctgggcgtcctctccgcccgaccgtacgcgccgaccggcgccgtggggcgggcgcgcatcgaccgccccgccgcccccttccccgaatcggagtgatccctcatgcagaggcagcacgccagcatcaccgatgccgcctacgggcagcgccgcagcgagataggcgcgctgtcggccggcctgacgccggacgaccccatcccccttgtggagtacaccgactgggagcacgaggtgtggcggttggtctgcgccgacctcgccgtccggcaccgcgtcgacgcggccgccccctacctccaggcggcggaggaactggccgtccccctggaccacgtcccgcaactgcgcgacgtcagcgcccggttggcgtcgatgtccggattccggctccagtccgccgccgcgctcgtcccgctgaaggagttctgcggaagcctggcgaattccgtcttccgctccacccagtacctccggcaccctcgctcgcccctctacagcgaggaccccgacatgctgcacgacctcgtcgggcacggcatcgccctggcgaacacccgcttcgcccacctctaccggctcgccggggaggccgcggcccgcgtgcagagcgccgatgccctccagttcatcggcaaggtgttctggttcaccctcgagtgcggtgtcgtccgcgagcacggtgaacgcaaggcgtacggggcgacgctggtctcctcgtacggtgagctcgaccacttccgcagcgcagcctttctgccgctggacatcgagagtctcgtcgacatcgagtacgacatcagcacgtaccagccgctgctgttcgaggcggactcgctggaccaggtcgaggacgtcctcggcgccttctgggggagctgcgacgacgagagcatcgcggccctgctcgacaggaggtcccgcagggtcggcagcaggcactgagcccggccctccgcctccgtacaccgggggcgagggcgcgtgtacgggagcggcggtttcctccccgccgccgctcccggtacgtccggaccgtggaccggacccggcccctcggtccttcaggtcctcaccgcgccgcgcgcaccacgtccgccacgatcgccacggcggccgggacgtccgccggaccgaggccccgatgggtcactgcccggatccgcccgtgcccgaactcgcccatggcgaggccgcgttgccgcgcgtcttccaggaagcgggcggcgtccagaccctcggccgtgacgcggaagaggacgatgttggtggtgacggagcccggggcgacgtcgatcccgtccacctccgccaggcccgccgcgaaccgcgccgcgagccgatggtcctcggcgagccggtcgaccatgtcggtcagcgcgaccgtaccggccgccgcgaacacgccggcctgccgcatgccgccgccgagcatcttgcggacgcgccgcgccttcccgatgaactcggccgatcccgcgaggatcgagccgatgggcgccgacagacccttggagaggcagaactggacggagtccgcgtgggcggcgatctcctccgccggcaaccccgacgccacggcggcgttgaagatccgggcgccgtccatgtgcaccgggacgccgtgcacggcggcgaaggccttgagctcggccaggtacgcctggcccagcacgcggccgcccatccggttgtgggtgttctccacacagatgaggcccggcagcgcgaactgggggtcgtccgggtcgggcgggaaggccgcggccaggtcgtccagcgcgagcgtgccgtcggggcgggtggggatcggctcgtagaccatgccgccgcagacacttgccccgccggcctcgtacaggtagatgtcgctctcgtcgccgacgagcaccttgccgccgcgcggcacgtgcacgagcagggcggcgaggttcgccatcgtgccgctgggcatcaggcacgcggcgggtttgccgacgctcttcgcggcgagttcctccaggtggttgacggtggggtcctcgccgtacacgtcgtccccaagggtcgcccggcccatggccgacagcatctcctcggtgggcagggtgaaggtgtcgcttcgcatctcgatcatggcagcccgtcccggctcagtcgttcgtcaatcggacagtgatgtgctccagcgccgcgtccagcgtccggtcgagctccgccaccgagtcggccgacgcgatgacgtgaccgatccggtcgtaggcgtcggtggccggacggatcgggtcgccggcgcggcgcgtgacgaggacctcggccacccccggcagtcgccgggcgggctcgacgccctccaggcccgcgagccgcccctcggcggagccggtgaggaaggcgacgccggtcgggatcagctccgtccgcggcagttcgacgggcagctcggccgccgcgcgcagttgctgggtcagcaggtcgggcccgccggccagcctgatcagctcgggaatcatgccgcctgcgagccgggcgttgatctcgatgatcgtcggccccttcgcggtcaggcgcacctcggtgtggcaggcgccgtgccgcagcccgaccgcctcgatcgccgcccgcaccatccgctcgatcgcgcgcgagccggccgtgtccagcggtgccggaaaggtgtgccggagttcgacgaacgagggcgggggcgacaccgacttccgggtgatgcccacgacgtgcaactcacccgccacgaagatcgtctccacgctgtactccggaccctggacgtgctcctcgacgagcacctccggcgggaccgcctggtcgcgcacgttgtgcgtgatcgccagcagcttcgcggcgtggtcgcgggcctgctcgacggaggtgcacagcagcacgcccgtcgacgccgagtccgaggccggcttgacgacgcaaggcagcccggtggccgcgaccgcgtcgggcatgtccgccacccgcgtcaccggcaccgagaccggctgtggcagtcccgcgtccgtcagcagccggcgggtcgccgacttgcggcggcacgcggcgacggccgcgggcgggttgccgggcaggccgagcgaggcggccagccgggcgacggcctccagatagaactcgctggtggtcgtcaccccagccacctcgccgggggcgaagtgggtacgcagggccgccgccagggcgtccccgtcgttggtgtcgcagcggatgacctggcagtcggcctcgccgatgccggggtagcggccgggccggccggtgagcagtacgggtgccagcccgaggtccctggcgcgcgcgagcgccagcatgccggtgcccgtcgtgttcgactcgacgaagaccaggcgccgccggggcgttgacggcacctcggcccgggcccagccgtccacctcggtgccgtagcgcaccgtggccggtgccatccgcagcgggaggccggcgagtccggcacgtttccagtaggcgtcgtcgtagatcgaatccacatagcgatccccccggtcggggaagatgccgacgacacgtgtgccgggggcgacggtgtcggccaggtgtctcagcacccggtagaccgaccccgaggaatttccggcgaacagcccttcctcctgggccagttcgcgggtcgcgacgaaggcctcccggtcgttcagccagtggatctcgtcgatctccgcgtagtccaggttggccgggatcaggctgttgccgatgccgctctgccgacgtcccggctggtcgggctggccgaacaggacgctgccgacggcgtcgacgccgatcacccgcagcggaccggagcttcccgcggcctgcagagcgtggcgcagcgcgcgggcggttccgcacagcgatccgccgctgccgaccgcgccgacgagcacgtcgatccggcccaggtccgccaccagttcgtcggcgagggcggcgtacgccagggggttctgcggattggagtactgccggggccagaacgcccccgggtactcggcgcgcagctcggccagccgctccagccgggcgctctgccagccgttcgcggtcatcgcctcgaccacgtgcaccgagcagccgagcgcggtcagcttcgcccgcgtgatcgcgtcgatccgggggtccgtcacgatgtgcaccggatggccgagggcgtggcccgccagggcgagccccagggccatggtgcccgaggagctctcgatgatcggcgcgccgggggccagaaccccgttcgcgcgcgcttcgagaactacctggcgggcgacccggtccttcatcgcgaacaggttctgcagttcgagcttggccgcgacggtcacgtccgagcgtgccgtccgcagccgcacgacgggcgtgtgcccgacggcctcgacgaggtcattgaagatcattgctggtccgcttcctgtcagctcgacaccaaggtctggtaacagagcacccgttcgcgatggacgagctgaccgcaccggttgatggcctcggccagccggctccggaaaccggggacgtcgtgcggcagcagcagcccgatcgtggacccgctgtgcgcggtcaccaccccgaccccgccgacctccgcgctcagcgccgtcatcgcgttcagcgtccgcttccggcagagtcgctggttgaggtgggcgctgcgggtcgccacctgcccgatggccgccgcgtcaccggcccgcaccgccgtccggatcctgtccagcagcagggcgtactcgtcccgctccgcgtcggtgaagttcttggggatccggttgaacgcgagcgtgtccacggtgccgccctcgtcgatgccgacgatggtcatcggcggcagggcgccgagcctgcccagcagcctgacctcgcggtgccggaacgccaccgcctccggatacatcacgccgtctgtcggctcgatccggcgcagcacgtcctcgatgacccggggcggcagctcgacgccgaccgcgctcgccacagcgcgcgccgtcgccaccagatcggccgacgaactcgccaggcctttgccctccggcagcgcgccgctgagccgcagcgtcccgccgccgtcggcgtaccgggcgagcacggcctcggcgacctggcgggccttcgtcttcgtcgccggggacacctcgacggagtcgtcggcgctccggtactcgaacgtcgccgtggcccatcgggcgatgggcagggtgaccaggaagtcgggtccgccgtcgggcagggcgccctggaggagctccccgaaggtaccgaaggcggagctgacggcgacggcgcgcgccggtgtcctcccgcgcccggccggcgggccgatgagctgccggctcgtcatgcggcgcccccggccccggacgagcgggcggcgtcggcggccgggggcgagacggcggcgtcggtggcggcgagcgcgtcccggaccgcggcccggcgcgtgtcccactccgcccggagcgcatcgatccgcgtgagctgctcggccagcagcgccgtcatcgcgtccggactcgtcgagcccgcggacaccttcgcgcgcagttgcgcgtccacgtccgcggagtgcgtcaggaacgaggccgggtcgtccagcggatgccccgcctccagagccgccttgccgagcgccgccggactgctgtgtcccggaagcccgtcgccctcggcgagtaccgcggtgacgtaccggccggcgacgacctgcgcggtacgccacggcaacccggcccgcagggtcagctcgttggccaggccgaagcccccgaagtggtcctcctcgcagacggcgcgcatccggtcggtgcgccactggagccggtcgaggaccagggtgaaaccggtcagtaccgcgcgcgtcgcgccgaacaggttgctcgcgtgcaggccggcctccttggagacctccaccatgttgctgtacggcgtgttccgctggccggcggcgaagtcgacgtagaaggccgtgaggtgcgcggtgcgcccgcgcagccgctccagcagcgggtagttcttcttctgcggcatggccgcggagatgcctgcgagctcgtccggcagctcgaccagtccgtacgcgctcgacgaccaggccatgaggtcggtgaggaagcggctgaaccctacgcccgccgaggcgaggtcggcggcgacgtcgagcagccattcccgcgaagcgaccgcgggcagcgcgtgcgggaccggtccgtcgcagccgattgcccgtgccagccaggcacggtcccagctcagttcctgcccggccatcggacctgcgccgagcggcgagcggttgatccggtcgtacgtgccgagcagccgggacgacacgctcagcgcgtgctccaccacggcgctgaggtagaagcccggcgtgatgatctgcgccgactggaggtgcgtgtacccgggcatcggcgaggtgatgtcgcgcgacgcccgttcgtgcgcgaccgtggccagctctccgagcagggccgcgatctcgctcacctgctcgcgtccgtaaagaagttgggccgtggcctggaggtcgttgcggctgcggtcgacgtgccaggcgggcacgggctccggcagggcccgggtgacgccggtctccatcgccagcgcgatgtcggtgagggccgccccggcgccggcggtcagccgctccggggtcagcccgtcgagcgccgccgcgagtcggtggacggactcgtccgccagtacgccgaggcggcggtactcgcgcagcagcgccttctcgatcaggacgtaccagcgcagcaggtgggcgacctcgtgcgtgaactggggctccaggaactcctgccggatgaagtcgtccggcgtggccgcgagccgaccggtcagcttcaacgggtgctgccttcctcagcggccgcgagggtcgcggtgacgatctccgccgcggcggcggggtgactgcggacgagataacggctcggctccgcgaaccaggtgatccgcgccccggggagtacgtccgcgcagcgcgccgtggcctcgccctcaccgggagccgcagggatcgccacgatcgtcgcgggcaggtcgagggtcccggagaaggcgccgaggtaccgctccgcctcgcggaggtcgtgccggtaggcgcgctcgatcaactcgccgcggctcgaacgcgactggtcgacgtcggtgagcgcgccggcgtcacgcagccaggcgccgatgtcggtcgatccggcggcagctgttccgccaccggccggtccgccgtcggtgggctcccgttcgatcccggcggccaggaagaggtggcggggaggtgcaccggcctcccgcagcgaccgggcggtctccagcgcgagcgccacgcccgccccgtgcccccacagcgccacgggcagctcgatccggtcgaggatctcccgggtcagcgggccggcgacccggtcgactccggccagctcctcgtccggccgggcgaagtcgtggccgggcagctccaccgcgtacaccgccacgtccgcggcggacaacgcccgggccatggcctcgaagttgagcgcgttgcccgcctcgtacggtacgcagacgagcgccgtggtcgcgtccttcggcaccgacagcggctggagcagcggggcctcggccggaccggcaccctcggcagcggcggccagatcggccagcaccgggttggccatgaggtccacgagcgagatgagcccgccgagctgcacgacgagccgcaccgccgccagcgacccgccgccgtgggcgaagaagtcgtcgttgcggccgacctcgtcgagcggcaggcccagcacctccgcccacacggtggcgatccgccgctccgcggcggtccgcggcggcgtcacgctgttgccgctcgcactgctggtctccagctccgccaaggcccgcttgtcgaccttgccgttgtcggtgagcgggaactcgggcagccagcgcagcgtacgcggcaccaactgcgtcggaagccgatcggccagcagctcacggaccgtcggtatcgcctgctcggccgtgtagaagcccgcaaggcgcttgctcgcgccgtccggcatcacgatcacgcatgccgcccgcaccccggccacccgcaggagctgcgcctcgacctcgccgacctcgacccggaccccgctgatcttcacctgctcgtcccgtcggccgacgaaccgcagccgcccgtcggacagccagtgtccgtagtcaccggtgcggtagcggcgcagcccggggcggaccggatcgtcgccgaaggcctctgcggtgcgttccggatcgttgatgtagccccggccgacgcacaccccggagaacgtgatctccccgatgctgtggtccgccacagggagcccgtcctcgccgacgacgtcgacaaggacgttggcgatgggcacgcccacggtgacctgctcatcgtccgccatgccgcggatgacctcgtgtgtcgtgtcgtccgatgcctcggtagcgccgtaggcgttgaccacgggcacgtcgggacactgcttgaaccagcgggtgagcacctgccggctcaccgcctcgccggtgacgccgagcatgcgcagcgagtcgggcgcacggtcgccccgctccagcctgctgacgatcacgtccaggtagctggggacgagctggaggacgccgacattctccgctgccaggagggagaggagcgcggggacgtcgagcatcagctccggatcgatgatcacggtgctgccgccgacgaggagcggcgcgagcgcctgccacagagagatgtcgaagcactgggacgcggtctgggccacggcagtgcccgccgcgatctcgaacgtgtcgatcttcgccagcaggtggttgagcatgccggcgtgttcgcaggcggcgcccttcggcgcccccgtggagccggaggtgaagtagatgtaggcaagcgccccgtccccgacacgggcgggctgcgcctcgtcggctgctgccggagccagcgggagcgcccgtacggccgcctccttgagcgggcgctccgacacatcgtcctcgacaagggccagccggctcccgctgcggtgcagcaggtcggcgatccgctcgtcggggtaggccggatcaatcggcagataggccccgcccgccttgaagatgccgagcatcgcagccagccagtcgagcgagcggtggctgatgaccgacaccacgccctcgggccgcagcccggcagagagaagggctccggccactcggttcgcagcggcgtcgagttccgcgtaggtccaccgcgtgccacggtggacggccgcgacggccgacggcgtcgcccgcgcgcactcctcgaagatctcgtgggcgcggcggtcggggagcggccgtaccggccccaccccgtgtgcctgccgaccgcggactgcctcggccttctccgtcacagtgccagcctttccggccgaacgataggggcggcctggattcctgagcggtaaccgatccgaaaggggagaggggggcgcggcgtccgcgcggcccggtctctcacggaaacacgctagtgagctgtggggttcgcccgtactgacatcggtcagggatccgccggcccgacgtactgacagatgccagtaccggtgggccgcccaccgctctgcatactcgacactcgctgcctcagaagaaggagacccggtgtttccgctcagcgccgcacagcaaatcgtctggctccagcagcaggtgcttccggagagccgcgcctatcacgccaccgcggtggtcgaatttcatggtgaattcgatccggtggtgatccgccgatgtatcgccgacgcggtcggccgccacgacgccttccggatccggatgtgtgacaccgattccgggatccccgcgcaggaggtcgtcgcggatatctccgtggaggtctcccagtacgacctgcgcgacgccgacgaccccgcggtacggcggggggaactgctccgcgggcaggtcagcaccgccttcgacctacggaccgcgccgctcgtccgctggatgctgctgcacctggccgacggtcactggcaactcgccatgaccgaacaccacctggtccacgacggccggtccaccgtgatcttcctcggcgacgtgctcgaccagtacgcggccgagatgtccggcggagaccacgtcccggaggctgccccctcgtacgaggagtacgtcgcccacacgggctcggacgagtaccgtgcgcgggtcgccgccgacgtcgcctggtgggcggagcggctcgacggtgcccggttcagcatcgacttccccaccctggggacccggcgctcggccctgttcgatcaccgcggcgggcagttccggcaggtgctctccgccccgctcatggaccgggtgcgggatgtcgcccaggagagtggtcacacggtcttcgccacgctgcttgccgtctactccgaactgtgccgccgccactccgggcaggacgaactggtcatcggcatgccgctggccaaccgcccggtggagttcgagcacacggtggggatgatggtcggcgccgtaccgcttcggctggcgatcgaccccctggctccgggcagcgacctcgccgaggaggccatgacggcggtcttcgacgccatcgaccatgagtcggctccgatccaggacctggtgacggcgctcaagcgcagcagcaaagggctgggcaacccgcttttcaacatcatgttcgccatgcacgacgccccctgtccgcccgtgaagatccccggcctctcggtcaacatggagatcgccgtgagcgccggcagcaccaagttcgacctgagcgtcgtggtcatgccggacaaggtcctgcaggcggaccacggcgaccacggctacgaactggtctgggagtactccactcagatgttcgggcccgaggacgtggagacgctcgccaccggattcgagaccctgctccgcgcctacgtcgccaggccttccgcgccgatcggcaccttggcaccggccgtggccgcgcgtccggcacgcgacgcccgcgacaaggacgaggagttcggtgcggcggaggtggcgccgcgcgccggggacgctccggccaccgacgccggaacgccttccggctcgctgtggctgcaggcgttccggcacatcctggagcgcgacgacatcgacgaggacaccgacttcttccaggcgggcggctattcgctgctcgtgccgctgctggtggcgcactacgagacgctcgcgggccgacggactccgccgagtctggtcttcgagttctcgttgccgcgagaactggaggcggcgacggccgcgatggcggggcgctgagccatgaccacgtaccggcacaccgtcgaggacgcggatgtcttcagcaaacacggcatcgagctgacggtctacgggcaacgcgacccgtcggccacggttgtgcgcgtgcaggtggaacgagggcatttccaggagttctccaattcccgaagttcctacatctattacatcgtcagcggtcggggggtgttccacctgaacgacgaggcgatcgccgtcggtgccaccgacctggtaaccgtcccgccgaacacccggatccactatttcggcacgatggagatggtcctcactgtggcgccggcattcgatgaacgagacgaacgacatatcaggttcgtcagcgagagcgagattcccgattgatgcccgtcacacccgctggatggaggatggcaagtcgatgaccacggaccacgccgcactgcccacggggtgccacgcgcgcactccggctccgccgccggacgcagcgtccctgccggacgatccgcccctgccgcacgaactcgccctgccgacggaccggtcgcggccggcccaccccgcgccggccgtggagctgcaccggttcgacctgactcccgggatccaccgtgccctgctcgccaccgccggggccgcccgggcgtcgctgcctacggcgctccatgccgccgtggccgctctgctgacccggctgggggccggcgtcgacatcccgatcgcggcaccggcggactccccggcccggtacctcagcctgcggatcggaacagacggggacccgagccttcgtgagcttctcgtacgggctcgggaggcgggtcgcacggcccgcgcgaggcaggacgtcgccacgcgacgccggacggacgacgccgacccggtgcggcgcgtcggaagcggtccggcggcccaggtggccgtgctcgtcgtcgacgagcacggccccggctgcgacccgacgggcacgaccggcttcgacctcgccctcaccgcgacggagcgacggggggccgagggcgaaccggccggcatcgcctgcgcactcgcctacgactccgagctcttcgaccccgggacggccgctgcgctggcggcgcgtctggtcacgcttctcacggcattcgccgacgtcccggacaccgcgctgtcgcgcgtggagctgttctccgacgacgagcgccgggcctggctggcgatgtccagtggaaccgagcatgcgatcggtgagtgcaccctggtcgagctgttcgagacacgggtccgggcgacgccggacgccgtggcgctggtgtgcggcgaccgttcgctgacgttcgccgaactgaacgggcgggccaacgccctggcccggcggctgatcggggcaggtgtccgctccgaggagccggtggccctcctgatggaccggtcggcggagcagatcgtctcgatcctggcgatcctcaaggcgggcggttgctacctcccgctgcacctggcgcatccggcgcgacgcatgaccggcgcccttgaggctgctgaggtcaggatcctgctgaccgatggttcgcacgccggccacgaggtcgcgagggccgccgggacgacactcctcgtgacggcggacggtccggccgcggcggacggcggtgacctcgaccgcaagccgctgcccgagcaggccgcgtacatcatgttcacctccggctcgaccggcacccccaagggcatcctggtgccccaccggagcgtggtgcacctggccctcgacagatgctggggcgaaggcgtgctggagcggatgctggtgcacttctccgccgcggtcgatccgtcgacgggcgagatctgggccccgctgctcaggaacggcagtctggtgatcgcaccgcccggcgatatcgacgcgcaggagctgcgggagctcgtctcccgctacggcgtcaccggcgccatcttccccggcgggctcttccggatgcttgccgacgacgacccggccgcgttcgcggggttgaccggcgtctacacgggcggcgaggtcatttcgccggtcgcggtgcgcaaggtgctcgacgcggctcccggtctcctcgtgcaccccctgtacggaccgaccgaggcgaccctggccgttacctaccacacgattcggcaggcaggggagctggcgggagatgtccccctcggccggccgatggacaaccggcacgtctatgtcctggacgagcatctcaacccggtgccgcccggcaccgtcggcgagctgtacctcggcggtgcgggcctggcccgcagctacgtcggcagcccggttctgacggccgaacggttcgtcccggatcccttccaaggggtgggtgcccggatgtaccggtcgggggatctggcccgctggacgcgtgacggcgtcctcatgttcgtgggccgcaccgacgagcaggtcaaggtacgcggctaccgcatcgagctcggggagatcgagaccgccctggcccggcaggaaggcgtccggagggtcgccgtcgtcgtccgggaggaccagcccggcgacgaacgactggtggcgtacctggtgccgggcgcgggagcggcaccggacccggaggcgctggccgaggagctgcgcgccactctgccggcgtacatggtgccctccgccttcgtcgccctgccggagctaccgctgacgccgaacgggaagacggaccgtacggccctgccggcgccggactacggcggcggcgcgggccaaggcccccgcacggccgacgaggagcgtctgtgcgctctgttcgccgaggtcctgggggtggaacgggtcggcgtggacgagggattcttcgccctgggcggggactcgctgttggcgacccggctgaggaccaggattcggagcgcgctcggtgtcgacctcagggcgcgagtgctgttccggcacccgaccgtcgccgagctcgcgcggctgctctgaccgcgcgcagtagtccggggaccacccggactactgcgcggggtcaccgaggtagccggggaagcggccctcggggtcccgggcggcacggatccgccggaatgccgaccaggcggcgtccgacatgatccggtccgcccggacggcgaggtcgctgtccccgaggtagcagccgaccgagtgaggcgccaggcggctcatcgtgcggtcgagccacgtccggctcaggacatcgtcggcgggggtcgtgccaatcgcgtacgcggcgaagtagaggtcggtctgcagcgacaccgccatgtccggggggcggcgggcgaccagcggcgtgaagtcgcccaggaccgtgaacgtcctgggcgtgggcagctcggtgaaggcgggcaccagcgccggaaccagctccgacgcggaaccggagaggaaggcgttgtccgcggcgtaccggtggttctccggattgccgcgcagctgctccgcctggagctccgcgaagtccaccggctcggcgaccgtgcgtgccgaggccctggcgaccaccggagacgaatcgagtgcggccagcgaggccgggccgccgtcgaacgacacggcgtcgacggtcagtaccggagcgtcggagccgggcggcgtggagccgacggcggccagctcgaccgacgccggcaggtcgtggcgggccacgtggtaccagctcaggacctccgcggcgagctcggaggggaagacgtacgcagaccgcgtcagctcccggaagcggggacgggtccgcagccggaaggcggtgaccactccgaagaatccgggccccgagccgcgcgccgcccagaacagatcggcgttctccgtctcggagcaccgcaccacctccccggcggcggtcaccacctccatggacacgagggactcggcggcccagccccagccgcggcagttccagccgataccaccctggagcaggaagcctcccatgccgacgctgggggagtggcccacgggaaagaaccggccgtgcccggcgagatacgggtccaggtccaggccgccgcgtactgccgggcccacggtcacggtcgcgtcggcggggtcgtaggacatcccggtgaacagcgcgaggtcgatgagcagggtgtcctcgcgcagtgaccaggcggcccaactgtgcccgccggaacggacggcgacccgccagccctccgccgctgccagcctcaccccctccgcgacgtcggtgacgtcggcggcccgcagcaccgctgccggacgccgcgagggcagccggcggttgaagacgcgtgcggtcgcggcatcggcgaagccggggtcgccgctccgccagaaggccccggtgaaagcgttcatcctcgggtggccccgtcctcgtcgccggacggaccgcggcgcaggctcgccggccgcatgtccgtccaggaacggccgacacgggccaggcagtcagccctcgtgccccgctgccccacctcgaaccagccggcgggcagatcctgcccggccggccagaccgagtactgctcctcgccgttccgcacgatgcggaactcgcctgcctcgtcgtcggacatgccgctcctcaccgtgcgtctgctgggagtacgaaccgctcggccgcttccaggagctgttccacggccttgcccgggaagcggtcctcgttgtagtgcgcgacgagctccggacccgtctcgtacaggttccacgcgacgaccacggtttccaggaaccgtttcccgccagggacgtcgagttcgacgtactccgcctcggtgccggcgaaaggcggcaggtcgtgcgaggagggcggcgcctcgttgagactgacgtacagcccggcctgccggtccggcaccatcagggtctcgctccagtaccgtccggcgaccagcagcggaacgctgtactcgaagacgtcgtgggtccggtggaagacctcccgggccgcctcggccgggctcttgtgcggtgtcttgaggtgcagcggcacagtctggacgaacagcccggcggtctgcgacgtgccgggcagcatccgaccgtgctggttgacggagattccggccaccggatcgccggtgacctccttcgcggcggcgagcacgccggcggtgaccgcggcgaagggggtcgcccgggcctccagcgagagcgcgtgcaggcgcgacttcgcgtcggcaggcagcacacggctgatcgtcctgggctggtaagcgcccgtggtgtcgccgccgaccgggaagggcgcggggaccgtgccgaactcgtcgacgtaggagcgccagaacgcgcggcactccttcccccacccgccggcgaacagacgccgctcctcggaggcgaagctctggtagctgccggcggccgtgacatcgccggaatcgccggtcagggcgcggcggtagaactcggtgaagtccgcccggatgagggcccatgaggccaggtcgttgatgatgtggtcgatcgcgatcccgaacaggtgcctgcgctcgccgcaccgcacgacggcgacccgtgagaagctcgggccgcccaggtcgaaggggcggccgatgaagcggcgcatcagctcgaccgcgtccgcgtccgacgcggcggtatggaactcgacctcgttgagcgcgtctgggtcggtgcgcgcctcctccggcgagagataggtgcggcgcagggcgtcgtgccggaggcacacccgccaccacgcgtcgcggagggcggcgacgtccagttcgccggtgagccacatcgccatgtagtgaaggttgtgccaatcggcgaactcgccggtcagccgggccatctccgccagcgaggtggggccctgagcggcccgggtcccggacgccgtcacttctcgccgccgtgcaccgcgccggaatccccctgcgcgaactcggcgtcgaggaaatcggaaaggctgcgcggcgaggcgtacgagaatacgtgacgcagcttcacgtcgataccgagggcgtcgtggatcctgccggtgatctgcaggacctgcaacgacgatccgttcttctcgaagagatccgcattctcgtcgagggcgggatctccgagaacctctcgccagatccgggtcaggaccgcgacgcgttccggcgcctttgcgttctgcagactcatatcgggagctcctcacggcgactgcgcgattctctggtgcccacaacgtgcagggttgcggccgagccgcacgctaccgatcttcggacagcgcccgtactgacaagagtcagggtgacgcaggggctacaccagcacactcacctggcaataagaatggtcggactcggtcgcggccaccgtcgtgctgagcagccgcagtgcccgcccgtagagaatgtggtccttctgtccgcccccgggggtcgtgggggtggcctcgaaggcgctccggtagtgcccggggcccaggacgtccccgagcacctcgcctatccgcccgtgattcgcgtcgagggcggcgaaggctgtccccgtgccgccgacggccagcaggtctgccgtgagcatggcccacaccggcgcgaacgccggctcggtggcgctcgcgccgaagcgcctcagagggaaacagtgcccgttgacgaacccgagcatccggtcgccgagggcgatcgacccgaccatgtagcccttgtcgtgaagggtccagcgctcgccccgcgggccggtaccgaccagctgtggccggggaaaacgtttgtacacggttttcgcgatcgggaaccgcgagaggatacccagggcgagggaagcatccttcgccatgtgtgaaacgctgagagggaaagacagtgagtgcgcatattcgaggcgcctcgccagatattccgactggctttcccggcggccgtcataatcatgcgcctcttgcagacacagaacgtcagggcggtgatccgccaggactgaggcgtagtaatcgagcgagggaatcccgtcgcgttggtgggattccccgaggatcccgccgcccatgttccaggtcgcgattctcagcagcgtaggcctcatcgatccgtcccagaaggtatggaaatgtacgggcgcctgtcggcatgccattttatgcgtctccggcaccggaccacactgacaggagtcagggtgccgcagcctcacttcgcgggccaagtggaaaagccgaacttcgcctccctccggaatccgtgcgctaggttgtccgtcatgattccggggatccgtcgacctgcagttcgaagttcctattctctagaaagtataggaacttcgaagcagctccagcctacatgaccacaccgtccttctgagctcggcgcgagcgcctgggtgaccgctgtccgcggtgggcgccgcaggctcgttcatcagtcgtccatcagacccttatcgcgtttccctacggttgcgggcgaggaccgagccgcttggggggaaccacatgctccgcatccacttcaatgacgcggatctggccaggacccggctcgcccccgctcccgacccgctgttcgaggtggccgcgagcatgcaccggctgcagtccggccgaggtcgctgggcctacgccgggtggtatcgggaggcgcggcgggatcttcgggagcaggggttggagcgggcgttgcggagtgttctgttgccgctgtatccgagggccgcttattacccggactttctgacgccgtcctccggggtggaggggctggaagcggggctggaggcgttgctggccacgccggcggagcgggtcgcggaggaggtcgggatgctggaccggctcatcggggcgccggggtgggcggggcggttgggcgagcaggaggtgcgtcgggagttcgtgggggtgctgcgggcgtatcacgatgcggtcgtcgtgccgcatcaggatcggatccaggcgcggatcgaggctgagcgggcggcacgggggcgggggctgctgcatggcggggtcgagggcatgctcgcggggctcggttccatgttccggtggtgtccgccggtgctggaggtcgcgtatccgcggcagacgcaggaccgggatctgtatctgaacgggcgtgggctcacccttgttccctcgtatttcaactggggtgagccggtcgcgttcgccgatcccgggttgccgccggtgctctggtactcgctgttgcacgagcctgcggcccgccccttgcgggaagaggatcctgagcggtctctggtcaatctgctcgggcgggcccgggcggtcgctctgcgggcggcggccggtggtgccacgacgggggagatcgcccgggcggccggggtttcggcgtccgccgccagtcggcatgccacggtgctgcgtgatgcggggctcatcacgactgcccgtcatggggcggctgttctgcatacgctcacccctgccggtgcgtctgttctgcgtgcggcccggagtgcggcgggcgaggcggctgtggacggtcgcgtcgagctgagctgacggatctggtcgcgccaccgctcttcgggtggtgccccctgtccactctggcgggggcgaagaacggtggcggaccgccggttccactgtcgcccggtcggggcgtgccgggccacactgttgcggctgggcgcaaaggctcaggtcagtgggtggttgccagggggcgggggtggtggtgggcggcgtgtcgtacgcgggtgagcagggtgtgggtgtcgaggcggtcggtgggggtccgggccaggcagtcgcggatgaccttctgccaggtgggcgggagtgcggcggacaggtggagctgctgggttccgcgggcgtagcgggttgccgcgtcgcagcgggcggccgtggtggtgccgggcagggggtgggtgccggtgaggagggtgtgggcgaggatgccgaaggcccatacgtcgaccgatggctgtgtgcgggcgcctcgttcgtccatctcgggccagagttgttcgggcgcggtgtggtcgcggctggtgaaggggggtgcgtaggcgtgggtgccttcgaggcgggcggctgtgttgaagtcggcgaggcgtacggttccgtcggccatgacgaggacgttggccggtttgaggtcgccgtggatccagccggcgtcgtggaggtgggtgaggccttcgcagatctgggtgagggtcgttccggggtcggtggggggtggtgcggtgttcaggcaggagtgggcgcgttcgaggatgagggcggtggcgccgtggagttgcgggtgccgggggtcgcgggcggtgagggtgtcgtacaggcggatcagccggggtgagcggaggtgttcgaggagttcgacttcgcgttggaggaggctgtgcagggggtcggggcgttggggggtgcggggggtggtgggccagaacttgagggcggcggttcggggggtgccgtgggtgcggtgtgcggcgtacacggtggtgaaggtgcctgaggcgaggggttcgtcgactttccagtcgccgatgcggtagccgtgggggacggtgacggtgtgccggcgggttctcatccgcatccctcgtaggcgtgggaggccagcacgatgaggtcgtcctcgcgtacgaggtcgaagcggagggcgagggaggcgagggtctccttcttgccgttggtgcggtgtccgggttcggcggtgtcggggcgggggcgtacgcgcagtttgagggccaggtagtcgatgctccagtagacggaggagcggttgacggtcggccaggtggggcggaggcgtcggacgaggtggtcgacggcgggggtgggggcgtggggttcgccgcggaggcggggttcgcagagggcggcgaggacggcgaagtagcgcttggtgcggtcgagggtgaaggcgggtgtggtggcggagccggggagttcccgggtttcggggccggcgaagagctggcggggggcccagacgtcgaaggtcaggaggtcgcctgcggcgggcaggacgacgcgggagaattcgaaggcgatgggggcgttgatgcggccgggggcgactttgatgtgttcgcccgcgccttcggggttctccacgacgtaggtctggtcggtgctgcggttggtcaggagccagaagtcgtgttctgcggtgatgttcccggcgatgcgggggacgccttcgtgggcgatggtgaggccgtcgggtgtttcccgtcggccgaaggtgaggctttcgccggcggcgatggtgatccggccgtccgggtgcgcgcaggccggaggtacgacgatgacgctgtacatggacttgtcccctagtcaagccatgagggccaccctcccccggtccaacaggggggagggtaggcgacgttgacgtacggggtaaagggggtgggggccggcgtggagtgggtgttcaggtgcggttcggggggccgatggtcagctccacgtcgtctcctctccgtgcgatccctttggcggcccaggtgccgtcgtcgatgagggtgccggccgcggtggtgtgggcggcggccatgaggcacgggtgtgccgtggggtgccgagcgtggtgccgggtgatgccgggtggtgccgtggggtgccgagcgtgatgccgggtggtgccatgtggtgtcgatgtggtgccatcctggggtgcgtggggtgcttctctggtgccattgagggtttagtggtggtgaagttgcaggtcaggggcgcgctctgagggtctgcgccaaagtggctcgacgtggtgccattcatgtgccatgatggcgtcatggacctcaccccctacgtcgacaacctccggcgggaactcgccgtcgctgcggatgccagcggtgacgaagcccgtgccctcgccgagcggctcagcgctcccctggagtccgctgcccggctgaccctgctcaacgtgctctccgaggccatgagcgacgtcacccgggagctggctcccggctcggtcgacgtacggctgcgcgggctcgatcccgagttcgtggtgacaccgccgccggcgcccgacccggtgcacgaggcgcgggagccggtcgtggctcccgtcgtggccgcgccgcccgccgcggagggcgacgacggcaccatggtccggaatccctatagtgagtcgtattatgcggccgcgaattctcatgtttgaccgcttatcatcgataagctctgctttttgttgacttccattgttcattccacggacaaaaacagagaaaggaaacgacagaggccaaaaagctcgctttcagcacctgtcgtttcctttcttttcagagggtattttaaataaaaacattaagttatgacgaagaagaacggaaacgccttaaaccggaaaattttcataaatagcgaaaacccgcgaggtcgccgccccgtaacaaggcggatcgccggaaaggacccgcaaatgataataattatcaattgcatactatcgacggcactgctgccagataacaccaccggggaaacattccatcatgatggccgtgcggacataggaagccagttcatccatcgctttcttgtctgctgccatttgctttgtgacatccagcgccgcacattcagcagcgtttttcagcgcgttttcgatcaacgtttcaatgttggtatcaacaccaggtttaactttgaacttatcggcactgacggttaccttgttctgcgctggctcatcacgctggataccaaggctgatgttgtagatattggtcaccggctgaggtgtttcgattgccgctgcgtggatagcaccatttgcgatagcggcgtccttgatgaatgacactccattgcgaataagttcgaaggagacggtgtcacgaatgcgctggtccagctcgtcgattgccttttgtgcagcagaggtatcaatctcaacgccaagcgtcatcgaagcgcaatattgctgctcaccaaaacgcgtattgaccaggtgttcaacggcaaatttctgcccttctgatgtcagaaaggtaaagtgattttctttctggtattcagttgctgtgtgtctggtttcagcaaaaccaagctcgcgcaattcggctgtgccagatttagaaggcagatcaccagacagcaacgcgccacggaaaaacagcgcatacagaacatccgtcgccgcgccggacaacgtgataattttatgacccatgatttatttccttttagacgtgagcctgtcgcacagcaaagccgccgaaagttcctcgaccgatgcccttgagagccttcaacccagtcagctccttccggtgggcgcggggcatgactatcgtcgccgcacttatgactgtcttctttatcatgcaactcgtaggacaggtgccggcagcgctctgggtcattttcggcgaggaccgctttcgctggagcgcgacgatgatcggcctgtcgcttgcggtattcggaatcttgcacgccctcgctcaagccttcgtcactggtcccgccaccaaacgtttcggcgagaagcaggccattatcgccggcatggcggccgacgcgctgggctacgtcttgctggcgttcgcgacgcgaggctggatggccttccccattatgattcttctcgcttccggcggcatcgggatgcccgcgttgcaggccatgctgtccaggcaggtagatgacgaccatcagggacagcttcaaggatcgctcgcggctcttaccagcctaacttcgatcattggaccgctgatcgtcacggcgatttatgccgcctcggcgagcacatggaacgggttggcatggattgtaggcgccgccctataccttgtctgcctccccgcgttgcgtcgcggtgcatggagccgggccacctcgacctgaatggaagccggcggcacctcgctaacggattcaccactccaagaattggagccaatcaattcttgcggagaactgtgaatgcgcaaaccaacccttggcagaacatatccatcgcgtccgccatctccagcagccgcacgcggcgcatctcgggcagcgttgggtcctgcagatccggctgtggaatgtgtgtcagttagggtgtggaaagtccccaggctccccagcaggcagaagtatgcaaagcatgcatctcaattagtcagcaaccaggtgtggaaagtccccaggctccccagcaggcagaagtatgcaaagcatgcatctcaattagtcagcaaccatagtcccgcccctaactccgcccatcccgcccctaactccgcccagttccgcccattctccgccccatggctgactaattttttttatttatgcagaggccgaggccgcctcggcctctgagctattccagaagtagtgaggaggcttttttggaggcctaggcttttgcaaaaagcttcacgctgccgcaagcactcagggcgcaagggctgctaaaggaagcggaacacgtagaaagccagtccgcagaaacggtgctgaccccggatgaatgtcagctactgggctatctggacaagggaaaacgcaagcgcaaagagaaagcaggtagcttgcagtgggcttacatggcgatagctagactgggcggttttatggacagcaagcgaaccggaattgccagctggggcgccctctggtaaggttgggaagccctgcaaagtaaactggatggctttcttgccgccaaggatctgatggcgcaggggatcaagatctgatcaagagacaggatgaggatcgtttcgcatgattgaacaagatggattgcacgcaggttctccggccgcttgggtggagaggctattcggctatgactgggcacaacagacaatcggctgctctgatgccgccgtgttccggctgtcagcgcaggggcgcccggttctttttgtcaagaccgacctgtccggtgccctgaatgaactgcaggacgaggcagcgcggctatcgtggctggccacgacgggcgttccttgcgcagctgtgctcgacgttgtcactgaagcgggaagggactggctgctattgggcgaagtgccggggcaggatctcctgtcatctcaccttgctcctgccgagaaagtatccatcatggctgatgcaatgcggcggctgcatacgcttgatccggctacctgcccattcgaccaccaagcgaaacatcgcatcgagcgagcacgtactcggatggaagccggtcttgtcgatcaggatgatctggacgaagagcatcaggggctcgcgccagccgaactgttcgccaggctcaaggcgcgcatgcccgacggcgaggatctcgtcgtgacccatggcgatgcctgcttgccgaatatcatggtggaaaatggccgcttttctggattcatcgactgtggccggctgggtgtggcggaccgctatcaggacatagcgttggctacccgtgatattgctgaagagcttggcggcgaatgggctgaccgcttcctcgtgctttacggtatcgccgctcccgattcgcagcgcatcgccttctatcgccttcttgacgagttcttctgagcgggactctggggttcgaaatgaccgaccaagcgacgcccaacctgccatcacgagatttcgattccaccgccgccttctatgaaaggttgggcttcggaatcgttttccgggacgccggctggatgatcctccagcgcggggatctcatgctggagttcttcgcccaccccgggctcgatcccctcgcgagttggttcagctgctgcctgaggctggacgacctcgcggagttctaccggcagtgcaaatccgtcggcatccaggaaaccagcagcggctatccgcgcatccatgcccccgaactgcaggagtggggaggcacgatggccgctttggtccggatctttgtgaaggaaccttacttctgtggtgtgacataattggacaaactacctacagagatttaaagctctaaggtaaatataaaatttttaagtgtataatgtgttaaactactgattctaattgtttgtgtattttagattccaacctatggaactgatgaatgggagcagtggtggaatgcctttaatgaggaaaacctgttttgctcagaagaaatgccatctagtgatgatgaggctactgctgactctcaacattctactcctccaaaaaagaagagaaaggtagaagaccccaaggactttccttcagaattgctaagttttttgagtcatgctgtgtttagtaatagaactcttgcttgctttgctatttacaccacaaaggaaaaagctgcactgctatacaagaaaattatggaaaaatattctgtaacctttataagtaggcataacagttataatcataacatactgttttttcttactccacacaggcatagagtgtctgctattaataactatgctcaaaaattgtgtacctttagctttttaatttgtaaaggggttaataaggaatatttgatgtatagtgccttgactagagatcataatcagccataccacatttgtagaggttttacttgctttaaaaaacctcccacacctccccctgaacctgaaacataaaatgaatgcaattgttgttgttaacttgtttattgcagcttataatggttacaaataaagcaatagcatcacaaatttcacaaataaagcatttttttcactgcattctagttgtggtttgtccaaactcatcaatgtatcttatcatgtctggatctgacgggtgcgcatgatcgtgctcctgtcgttgaggacccggctaggctggcggggttgccttactggttagcagaatgaatcaccgatacgcgagcgaacgtgaagcgactgctgctgcaaaacgtctgcgacctgagcaacaacatgaatggtcttcggtttccgtgtttcgtaaagtctggaaacgcggaagtcagcgctcttccgcttcctcgctcactgactcgctgcgctcggtcgttcggctgcggcgagcggtatcagctcactcaaaggcggtaatacggttatccacagaatcaggggataacgcaggaaagaacatgtgagcaaaaggccagcaaaaggccaggaaccgtaaaaaggccgcgttgctggcgtttttccataggctccgcccccctgacgagcatcacaaaaatcgacgctcaagtcagaggtggcgaaacccgacaggactataaagataccaggcgtttccccctggaagctccctcgtgcgctctcctgttccgaccctgccgcttaccggatacctgtccgcctttctcccttcgggaagcgtggcgctttctcatagctcacgctgtaggtatctcagttcggtgtaggtcgttcgctccaagctgggctgtgtgcacgaaccccccgttcagcccgaccgctgcgccttatccggtaactatcgtcttgagtccaacccggtaagacacgacttatcgccactggcagcagccactggtaacaggattagcagagcgaggtatgtaggcggtgctacagagttcttgaagtggtggcctaactacggctacactagaaggacagtatttggtatctgcgctctgctgaagccagttaccttcggaaaaagagttggtagctcttgatccggcaaacaaaccaccgctggtagcggtggtttttttgtttgcaagcagcagattacgcgcagaaaaaaaggatctcaagaagatcctttgatcttttctacggggtctgacgctcagtggaacgaaaactcacgttaagggattttggtcatgagattatcaaaaaggatcttcacctagatccttttaaattaaaaatgaagttttaaatcaatctaaagtatatatgagtaaacttggtctgacagttaccaatgcttaatcagtgaggcacctatctcagcgatctgtctatttcgttcatccatagttgcctgactccccgtcgtgtagataactacgatacgggagggcttaccatctggccccagtgctgcaatgataccgcgagacccacgctcaccggctccagatttatcagcaataaaccagccagccggaagggccgagcgcagaagtggtcctgcaactttatccgcctccatccagtctattaattgttgccgggaagctagagtaagtagttcgccagttaatagtttgcgcaacgttgttgccattgctgcaggcatcgtggtgtcacgctcgtcgtttggtatggcttcattcagctccggttcccaacgatcaaggcgagttacatgatcccccatgttgtgcaaaaaagcggttagctccttcggtcctccgatcgcccttcccaacagttgcgcagcctgaatggcgaatggcgcctgatgcggtattttctccttacgcatctgtgcggtatttcacaccgcataaattccccaatgtcaagcacttccggaatcgggagcgcggccgatgcaaagtgccgataaacataacgatctttgtagaaaccatcggcgcagctatttacccgcaggacatatccacgccctcctacatcgaagctgaaagcacgagattcttcgccctccgagagctgcatcaggtcggagacgctgtcgaacttttcgatcagaaacttctcgacagacgtagatcaggcttcccgggtgtctcgctacgccgctacgtcttccgtgccgtcctgggcgtcgtcttcgtcgtcgtcggtcggcggcttcgcccacgtgatcgaagcgcgcttctcgatgggcgttccctgccccctgcccgtagtcgacttcgtgacaacgatcttgtctacgaagagcccgacgaacacgcgcttgtcgtctactgacgcgcgcccccaccacgacttagggccggtcgggtcagcgtcggcgtcttcggggaaccattggtcaaggggaagcttcggggcttcggcggcttcaagttcggcaagccgctcttccgccccttgctgccggagcgtcagcgctgcctgttgcttccggaagtgcttcctgccaacgggtccgtcgtacgcgcctgccgcgcggtcttcgtacagctcttcaagggcgttcagggcgtcggcgcgctccgcaacaaggttcgcccgttcgccgctcttctcaggcgcctcagtgagcttgccgaagcgtcgggcggcttcccacagaagcgccaacgtctcttcgtcgccttcggcgtgcctgatcttgttgaagatgcgttccgcaacgaacttgtcgagtgccgccatgctgacgttgcacgtgccttcgtgctgcccaggtgcggacgggtcgaccaccttccggcgacggcagcggtaagagtccttgatcgattcttccccgcgcttcgaagtcatgacggcgccacactcgcagtacagcttgtccatggcggacagaatggcttgcccccgggaaagccccttgccgcgccccctgccgtccaaccacgcctgaagctcataccactcagcgggctcgatgatcggtccgcaatcaagctcgaccggccggagcgtgatcgggtcgcgctgaatgcggtaaccctcaatcttcgtggtcggcgtgccgtccggcttcttcttgtagatcacctcagcggcgaagcccgcaatacgcgggtcccgaaggattcgcataacggttgccgggtcccaggcgcttgaagcggtcttcttcccaatcgtctcgccccgggtcggcacggcgtcagcgtccatgcgcttacaaagccccgtgatgctgcccgggtgaatggcggcttgactgcccggcttgaagggaaggtgtttgtgcgtcttgatctcacgccaccaccaccggattacgtcgggctcgaactcgaagggtccggtaaggggagtggtcgagtgcgcaagcttgttgatgacgacattgaccattcggccgttgcgcgtgatctccttcgtctccgaaacaagctcgaagccgtaaggcgccttcccgccgacgtacccgcccaattcgcgctgaaggttcttcgtgtcgagaatcttcgccgacttcagcgaagattctttgtgcgacgcgtcgagccgcataatcaggtgaatcaggtccatgacgtttccctgccggaagacgccttcctgagtggaaacaatcgtcacgcccagggcgagcaattccgagacaatcggaatcgcgtccatgaccttcaggcgcgagaagcgcgacacgtcatagacaatgatcatgttgagccgcccggcgcggcattcgttcaggatgcgttcgaactccgggcgctccgccgtcccgaacgccgacgtgcccggcgcttcgctgaaatgcccgacgaacctgaaccggcccccgtcgcgctcgacttcgcgctgaaggtcggccgccttgtcttcgttggcgctacgctgtgtcgctgggcttgctgcgctcgaatttcgcgctcgcgcgactgacggtcgtaagcacccgcgtacgtgtccaccccggtcacaaccccttgtgtcatgtcggcgaccctacgcccccaactgagagaactcaaaggttaccccagttggggcactactcccgaaaaccgcttctgacctgggaaaacgtgaagccccggggcatccgctgagggttgccgccggggcttcggtgtgtccgtcagtacgggccatagaggggcgtcgtgtaacccacccagggcgattgctccggcacggggaagccgcgccacgccttcgggacgtctcaggtcgaggtggcccggctccatgcaccgcgacgcaacgcggggaggcagacaaggtatagggcggcgcctacaatccatgccaacccgttccatgtgctcgccgaggcggcataaatcgccgtgacgatcagcggtccagtgatcgaagttaggctggtaagagccgcgagcgatccttgaagctgtccctgatggtcgtcatctacctgcctggacagcatggcctgcaacgcgggcatcccgatgccgccggaagcgagaagaatcataatggggaaggccatccagcctcgcgtcgcgaacgccagcaagacgtagcccagcgcgtcggccgccatgccggcgataatggcctgcttctcgccgaaacgtttggtggcgggaccagtgacgaaggcttgagcgagggcgtgcaagattccgaataccgcaagcgacaggccgatcatcgtcgcgctccagcgaaagcggtcctcgccgaaaatgacccagagcgctgccggcacctgtcctacgagttgcatgataaagaagacagtcataagtgcggcgacgatagtcatgccccgcgcccaccggaaggagctgactgggttgaaggctctcaagggcatcggtcgacgctctcccttatgcgactcctgcattaggaagcagcccagtagtaggttgaggccgttgagcaccgccgccgcaaggaatggtgcatgcaaggagatggcgcccaacagtcccccggccacggggcctgccaccatacccacgccgaaacaagcgctcatgagcccgaagtggcgagcccgatcttccccatcggtgatgtcggcgatataggcgccagcaaccgcacctgtggcgccggtgatgccggccacgatgcgtccggcgtagaggatccacaggacgggtgtggtcgccatgatcgcgtagtcgatagtggctccaagtagcgaagcgagcaggactgggcggcggccaaagcggtcggacagtgctccgagaacgggtgcgcatagaaattgcatcaacgcatatagcgctagcagcacgccatagtgactggcgatgctgtcggaatggacgatatcccgcaagaggcccggcagtaccggcataaccaagcctatgcctacagcatccagggtgacggtgccgaggatgacgatgagcgcattgttagatttcatgacattgcactccaccgctgatgacatcagtcgatcatagcacgatcaacggcactgttgcaaatagtcggtggtgataaacttatcatccccttttgctgatggagctgcacatgaacccattcaagacgtcatggcaatcgctagagcttgcatgcctgcaggtcgacggatcttttccgctgcataaccctgcttcggggtcattatagcgattttttcggtatatccatcctttttcgcacgatatacaggattttgccaaagggttcgtgtagactttccttggtgtatccaacggcgtcagccgggcaggataggtgaagtaggcccacccgcgagcgggtgttccttcttcactgtcccttattcgcacctggcggtgctcaacgggaatcctgctctgcgaggctggccggctaccgccggcgtaacagatgagggcaagcggatggctgatgaaaccaagccaaccaggaagggcagcccacctatcaaggtgtactgccttccagacgaacgaagagcgattgaggaaaaggcggcggcggccggcatgagcctgtcggcctacctgctggccgtcggccagggctacaaaatcacgggcgtcgtggactatgagcacgtccgcgagctggcccgcatcaatggcgacctgggccgcctgggcggcctgctgaaactctggctcaccgacgacccgcgcacggcgcggttcggtgatgccacgatcctcgccctgctggcgaagatcgaagagaagcaggacgagcttggcaaggtcatgatgggcgtggtccgcccgagggcagagccatgacttttttagccgctaaaacggccggggggtgcgcgtgattgccaagcacgtccccatgcgctccatcaagaagagcgacttcgcgaagctggtgaagtacatcaccgacgagcaaggcaagaccgatccccggggacctgcaggtcgactctagctagctggactcaaccaagtcattctgagaatagtgtatgcggcgaccgagttgctcttgcccggcgtcaacacgggataataccgcgccacatagcagaactttaaaagtgctcatcattggaaaacgttcttcggggcgaaaactctcaaggatcttaccgctgttgagatccagttcgatgtaacccactcgtgcacccaactgatcttcagcatcttttactttcaccagcgtttctgggtgagcaaaaacaggaaggcaaaatgccgcaaaaaagggaataagggcgacacggaaatgttgaatactcatactcttcctttttcaatattattgaagcatttatcagggttattgtctcatgagcggatacatatttgaatgtatttagaaaaataaacaaataggggttccgcgcacatttccccgaaaagtgccacctgacgtctaagaaaccattattatcatgacattaacctataaaaataggcgtatcacgaggccctttcgtcttcaagaattcgcggccgcaattaaccctcactaaaggg

SEQ ID NO: 3 - DNA, 9436 bp, synthetic construct
  misc_feature 1..9436: note = pUWL201 derivative containing npsM from Streptomyces sp. DSM 5940 and pac21h, phhA from Streptomyces coeruleorubidus AB1183F-64
  source 1..9436: mol_type = other DNA
atgtcgcccttcatcgctcccgacgtccctgagcaccttctagacactgttcgcgtcttcctgtacgcgcgtcagtctaagggccggtccgacggctcagacgtgtcgaccgaagcacagctagcggccggtcgtgcgttggtcgcgtctcgcaacgcccaggggggtgcgcgctgggtcgtggcaggtgagttcgtggacgtcgggcgctccggctgggacccgaacgtgacccgtgccgacttcgagcgcatgatgggcgaagtccgcgccggcgaaggtgacgttgtcgttgtgaatgagctttcccggctcactcgcaagggcgcccatgacgcgctcgaaatcgacaacgaattgaagaagcacggcgtgcgcttcatgtcggttcttgagccgttccttgacacgtctacccctatcggcgtcgccattttcgcgctgatcgctgcccttgcgaaacaggacagtgacctgaaggcggagcgcctgaagggtgcgaaagacgagattgccgcgctgggtggcgttcactcgtcttccgccccgttcggaatgcgcgccgtgcgcaagaaggtcgataatctcgtgatctccgttcttgagccggacgaagacaacccggatcacgtcgagctagttgagcgcatggcgaaaatgtcgttcgaaggcgtgtccgacaacgccattgcaacgaccttcgagaaggaaaagatcccgtcgcccggaatggctgagagacgcgccacggaaaagcgtcttgcgtccgtcaaggcacgtcgcctgaacggcgctgaaaagccgatcatgtggcgcgctcaaacggtccgatggattctcaaccatcccgcaatcggcggtttcgcattcgagcgtgtgaagcacggtaaggcgcacatcaacgtcatacggcgcgaccccggcggcaagccgctaacgccccacacgggcattctcagcggctcgaagtggcttgagcttcaagagaagcgttccgggaagaatctcagcgaccggaagcctggggccgaagtcgaaccgacgcttctgagcgggtggcgtttcctggggtgccgaatctgcggcggctcaatgggtcagtcccagggtggccgtaagcgcaacggcgaccttgccgaaggcaattacatgtgcgccaacccgaaggggcacggcggcttgtcggtcaagcgcagcgaactggacgaattcgttgcttcgaaggtgtgggcacggctccgcacagccgacatggaagatgaacacgatcaggcatggattgccgccgctgcggagcgcttcgcccttcagcacgacctagcgggggtggccgatgagcggcgcgaacaacaggcgcacctagacaacgtgcggcgctccatcaaggaccttcaggcggaccgtaagcccggtctgtacgtcgggcgtgaagagctggaaacgtggcgctcaacggtgctgcaataccggtcctacgaagcggagtgcacgacccgactcgctgagcttgacgagaagatgaacggcagcacccgcgttccgtctgagtggttcagcggcgaagacccgacggccgaagggggcatctgggcaagctgggacgtgtacgagcgtcgggagttcctgagcttcttccttgactccgtcatggtcgaccgggggcgccaccctgagacgaagaaatacatccccctgaaggaccgtgtgacgctcaagtgggcggagctgctgaaggaggaagacgaagcgagcgaagccactgagcgggagcttgcggcgctgtagcgcacagcgggaggggtcgagccggcggacggttcggccccttttttggccttgaaatcgttagttaggctaactagaaaaaaaaaaggctccaaaaggagcctttaaactaggaccgggccccccctcgaggtccagcccgacccgagcacgcgccggcacgcctggtcgatgtcggaccggagttcgaggtacgcggcttgcaggtccaggaaggggacgtccatgcgagtgtccgttcgagtggcggcttgcgcccgatgctagtcgcggttgatcggcgatcgcaggtgcacgcggtcgatcttgacggctggcgagaggtgcggggaggatctgaccgacgcggtccacacgtggcaccgcgatgctgttgtgggcacaatcgtgccggttggtaggatcgacggtatcgataagcttgatatcatggacaaccttttcgagcgtgatgcagaagtgattctgacctggcgcgtccaggcccgccacctgggtggatccactacccaggaaaggatcaacctgaaggtcggcgatcggctggacttcggcatacccaacgccggcggagaattccagccccgtgcgacgcccagcatcggcacttttgaggtgtccgaccagcacctcttcttctcgaacttcaccaccagcaccacgttcgtcatcgagaatctggagggcgggaccgaactcgtcaaggcgcgcccccgccagctcggcatggtgatcccgttcgagatgtcgcgcatcctcatcccctccagcgcaagcatcggcgaactcaccgtcttcacatccccgccccgcctgctcgggcccgagatggccgccacgcccaccgagtccgcgatgtccaaactggacgcgacgaccaagtacttcgccgttctcgtcgccttgtgcgagccgcgtctgcgcggttcctcgatggcggctgtgccctccgtccaggaggtggtggaaagactgcggggggtcgagcagttcagggacgccaaccgcagcagcgtcaactaccacatcgactatctggctgaccagaagcttccggtcagccagtgggccaagtacctgaacgaagggcgcatgcattcgaagcgcgaggccctggtcgccttctcgctccgcttcgacctggtccgcgaggaacacctcgccctcctccccgacgtcaaactcctgcgcgcgcaacgatgtcttgaggcacggcaagccacgaaggtggcaacgggcgcgatctcatgaactagcctagtaacgctcactgggtaccagcccgacccgagcacgcgccggcacgcctggtcgatgtcggaccggagttcgaggtacgcggcttgcaggtccaggaaggggacgtccatgcgagtgtccgttcgagtggcggcttgcgcccgatgctagtcgcggttgatcggcgatcgcaggtgcacgcggtcgatcttgacggctggcgagaggtgcggggaggatctgaccgacgcggtccacacgtggcaccgcgatgctgttgtgggcacaatcgtgccggttggtaggatcgtctagaacaggaggccccatatgtctctcacattggtcgagcgattcctgcgcggactggaactatccccggacggtcccgcagtacggatcggttcggatgtcgtcacctatcggcaggtgcacaacaccgccttgcactgggcggaatcgctcatggcgaatggttctcctggttcggtaggcgtgctggcgggcaagagcaggacgtcctatgtgggccttctggcggtgctgtacgcgggcgccaccgttgttccgttgcagccgaacttccccgccgcactcacccgtcggatgatcaaggtggccggggtggacacactgatcgccgacgagcgcggtctggaggtcctaccggagatcaccgatcaggaaacggcggttcgagtcctcgacaccggcggtttcgccgacaggtttccgacaattccggtgacttcgcatccggagatttcggagccggtccgagtggccccttcggatccggcatacattctcttcacgtcgggctcgaccgggaccccgaagggagttcccatatcgcacggcggtttcgcgcactatttcgagcagcttgacaaacggtgcgacttccgcccggacgacgtgttcgcccagacctacgacctcaatttcgaccccggtatccacgacgtgttcgccgcctggggtgcgggcgcgatgatgcaggcagtgccgctgtcggcgtatcgggatcttcccgcatacctcgccgagcatggggtcacggtgtggcactccacgccgagcggtatctggatggcccgggagatgggtggtcttgagaaaggcgcgctgcctggcctgagatggtcgttcttcggcggggaggcgctgcgctgtcaggacgtcgcggactggctggcggctgcacccggatcaaagctggagaacctctacgggccgaccgagttctcgatcggcatctgctggcatcgctggtcgggcgaggagtccgaaaggcgtggcgtcaacggcacggtgccgatcgggaaggtgcatgacggcaacgacttccgcctggtgacggagcagggggaagagtcgtccgtggagggtgagctgtggatcacgggtccgcagatggcatccggatacctcgacccggccgacgacgagggtcggttcgtcgacttcgccggtcggcgctggtaccgcacgggtgaccgggtacgcgcgcatcccgacggtgaactcgtctacatcggccgcttggactcgcaggtgaaggtgcacgggtggcgcgttgagctggcggaagtggaccacgtggtgcgcgagtgcgacggggtgcgcgacgcggtcaccgtcaccaggcccgcgctgcacggcacggagctggtcgtgttctacaccggcgacgaagtgccggagcaggtgctggccgatggtgtgcgcgcggtgctgccgcacagcacactgccccgccgatacgttcacgtggacagtttcccgttgaattccaaccgaaaagtcgaccggatcgcgctgcggaagcgggcggaggagttgcctggctgagcgaggcgccgaccgggagagccctgagaggtcggctcgactggtctgcggaacgaaacgggatgcccgctaccacgaaagcaccctccatctgtaccgaagtcggaccggctacggagtttatgaagccacgttcctgccgactgcgaccggcgactggaaaatctctcgtgccgtgatcgaggggcatgctctgcgacatgccttcccaagttgccgagcaccatgtccttggcatttcttccgcctgaccgtgcgagccgactgccgcaatgaactcgatatcgcgccagcctctctcgccgccgcggaagcggacatggcgaaggcaggtattgcgggccggatgcgttcggccaggccgccgcccgctctcacacgatcgtcttgaattggagtgatccctcatgcaagggccgcacgcccagatgaccgatgccgcctacgaaatacgccgaagtgagatcgcggcactgtccaccgatctagcgccggaggatcccattccggtggtcgaatacaccgagtgggagcacgaggtgtggcggacggtctgcgtcgacctcaccgcccggcaccgcacggacgcggctgctgaatacctcgaatccgcagagcaattggccgtcccgctggaccacgtacctcaactccgcgacgtgagcggccgcttgggatcgatatcgggttttacttttcagtcagcccccgcgctcgttccgttgcgggagttctgcggaggtctggcgaattccgtcttccactccacccagtacctccggcatcctcgttcccccttctacaccgaggaccccgatctgctgcacgacctcgtcggtcacggcaacgtcctggccagcgaccgcttcgcccgcctgtaccggctcgcgggtaacgccgcggcccgcgtgcacagcaccgaggccctgcagttcatcggcaaggtgttctggttcaccctcgaatgcggtgtcgtccgcgagcgcggtgaacgcaaggcctacggggcgacgctggtctcctcctacggggaactcgaccacttccgcagcgccgacttccggccgctggacatcaagagccttgccgacgtcgaatatgacatctccacgtatcagccgatcctgttcgaagcggactcgatggacgaggtggaggacacggtcggctccttctgggacacgtgtgacgacgacagcatcgcggccctgctcggcgggacgtcccgctcggtgacacctcactgagccaagcttggatccaaaaaaaaaggctccaaaaggagcctttaagcggccgcgcgcgatatcgaattcgtaatcatgtcatagctgtttcctgtgtgaaattgttatccgctcacaattccacacaacatacgagccggaagcataaagtgtaaagcctggggtgcctaatgagtgagctaactcacattaattgcgttgcgctcactgcccgctttccagtcgggaaacctgtcgtgccagctgcattaatgaatcggccaacgcgcggggagaggcggtttgcgtattgggcgctcttccgcttcctcgctcactgactcgctgcgctcggtcgttcggctgcggcgagcggtatcagctcactcaaaggcggtaatacggttatccacagaatcaggggataacgcaggaaagaacatgtgagcaaaaggccagcaaaaggccaggaaccgtaaaaaggccgcgttgctggcgtttttccataggctccgcccccctgacgagcatcacaaaaatcgacgctcaagtcagaggtggcgaaacccgacaggactataaagataccaggcgtttccccctggaagctccctcgtgcgctctcctgttccgaccctgccgcttaccggatacctgtccgcctttctcccttcgggaagcgtggcgctttctcatagctcacgctgtaggtatctcagttcggtgtaggtcgttcgctccaagctgggctgtgtgcacgaaccccccgttcagcccgaccgctgcgccttatccggtaactatcgtcttgagtccaacccggtaagacacgacttatcgccactggcagcagccactggtaacaggattagcagagcgaggtatgtaggcggtgctacagagttcttgaagtggtggcctaactacggctacactagaagaacagtatttggtatctgcgctctgctgaagccagttaccttcggaaaaagagttggtagctcttgatccggcaaacaaaccaccgctggtagcggtggtttttttgtttgcaagcagcagattacgcgcagaaaaaaaggatctcaagaagatcctttgatcttttctacggggtctgacgctcagtggaacgaaaactcacgttaagggattttggtcatgagattatcaaaaaggatcttcacctagatccttttggttcatgtgcagctccatcagcaaaaggggatgataagtttatcaccaccgactatttgcaacagtgccgttgatcgtgctatgatcgactgatgtcatcagcggtggagtgcaatgtcgtgcaatacgaatggcgaaaagccgagctcatcggtcagcttctcaaccttggggttacccccggcggtgtgctgctggtccacagctccttccgtagcgtccggcccctcgaagatgggccacttggactgatcgaggccctgcgtgctgcgctgggtccgggagggacgctcgtcatgccctcgtggtcaggtctggacgacgagccgttcgatcctgccacgtcgcccgttacaccggaccttggagttgtctctgacacattctggcgcctgccaaatgtaaagcgcagcgcccatccatttgcctttgcggcagcggggccacaggcagagcagatcatctctgatccattgcccctgccacctcactcgcctgcaagcccggtcgcccgtgtccatgaactcgatgggcaggtacttctcctcggcgtgggacacgatgccaacacgacgctgcatcttgccgagttgatggcaaaggttccctatggggtgccgagacactgcaccattcttcaggatggcaagttggtacgcgtcgattatctcgagaatgaccactgctgtgagcgctttgccttggcggacaggtggctcaaggagaagagccttcagaaggaaggtccagtcggtcatgcctttgctcggttgatccgctcccgcgacattgtggcgacagccctgggtcaactgggccgagatccgttgatcttcctgcatccgccagaggcgggatgcgaagaatgcgatgccgctcgccagtcgattggctgagctcatgagcggagaacgagatgacgttggaggggcaaggtcgcgctgattgctggggcaacacgtggagcggatcggggattgtctttcttcagctcgctgatgatatgctgacgctcaatgccgtttggcctccgactaacgaaaatcccgcatttggacggctgatccgattggcacggcggacggcgaatggcggagcagacgctcgtccgggggcaatgagatatgaaaaagcctgaactcaccgcgacgtatcgggccctggccagctagctagagtcgacctgcaggtccccggggatcggtcttgccttgctcgtcggtgatgtacttcaccagctccgcgaagtcgctcttcttgatggagcgcatggggacgtgcttggcaatcacgcgcaccccccggccgttttagcggctaaaaaagtcatggctctgccctcgggcggaccacgcccatcatgaccttgccaagctcgtcctgcttctcttcgatcttcgccagcagggcgaggatcgtggcatcaccgaaccgcgccgtgcgcgggtcgtcggtgagccagagtttcagcaggccgcccaggcggcccaggtcgccattgatgcgggccagctcgcggacgtgctcatagtccacgacgcccgtgattttgtagccctggccgacggccagcaggtaggccgacaggctcatgccggccgccgccgccttttcctcaatcgctcttcgttcgtctggaaggcagtacaccttgataggtgggctgcccttcctggttggcttggtttcatcagccatccgcttgccctcatctgttacgccggcggtagccggccagcctcgcagagcaggattcccgttgagcaccgccaggtgcgaataagggacagtgaagaaggaacacccgctcgcgggtgggcctacttcacctatcctgcccggctgacgccgttggatacaccaaggaaagtctacacgaaccctttggcaaaatcctgtatatcgtgcgaaaaaggatggatataccgaaaaaatcgctataatgaccccgaagcagggttatgcagcggaaaagatccgtcgacctgcaggcatgctggcgccggacggggcttcagacgtttcgggtgctgggttgttgtctctggacagtgatccatgggaaactactcagcaccaccaatgttcccaaaagaaagcgcaggtcagcgcccatgagccaagatctaggc